European Patent Application EP 4 800 105 A1, published September 2, 2026. Title: 一种高效低脱靶的基因编辑工具. Applicant: 石药集团中奇制药技术（石家庄）有限公司. The sequence listing filed with the application follows.

SEQUENCE LISTING (91 sequences)

SEQ ID NO: 1 - DNA, 4555 bp, synthetic construct
  source 1..4555: mol_type = other DNA
gggagacccaagctggctagcgtttaaacttaagcttggtaccgagctcggatccactagtccagtgtggtggaattcgggaaataagagagaaaagaagagtaagaagaaatataagagccaccatggccccaaagaagaagcggaaggtcggtatccacggagtcccagcagccgacaagaagtacagcatcggcctggacatcggcaccaactctgtgggctgggccgtgatcaccgacgagtacaaggtgcccagcaagaaattcaaggtgctgggcaacaccgaccggcacagcatcaagaagaacctgatcggagccctgctgttcgacagcggcgaaacagccgaggccacccggctgaagagaaccgccagaagaagatacaccagacggaagaaccggatctgctatctgcaagagatcttcagcaacgagatggccaaggtggacgacagcttcttccacagactggaagagtccttcctggtggaagaggataagaagcacgagcggcaccccatcttcggcaacatcgtggacgaggtggcctaccacgagaagtaccccaccatctaccacctgagaaagaaactggtggacagcaccgacaaggccgacctgcggctgatctatctggccctggcccacatgatcaagttccggggccacttcctgatcgagggcgacctgaaccccgacaacagcgacgtggacaagctgttcatccagctggtgcagacctacaaccagctgttcgaggaaaaccccatcaacgccagcggcgtggacgccaaggccatcctgtctgccagactgagcaagagcagacggctggaaaatctgatcgcccagctgcccggcgagaagaagaatggcctgttcggaaacctgattgccctgagcctgggcctgacccccaacttcaagagcaacttcgacctggccgaggatgccaaactgcagctgagcaaggacacctacgacgacgacctggacaacctgctggcccagatcggcgaccagtacgccgacctgtttctggccgccaagaacctgtccgacgccatcctgctgagcgacatcctgagagtgaacaccgagatcaccaaggcccccctgagcgcctctatgatcaagagatacgacgagcaccaccaggacctgaccctgctgaaagctctcgtgcggcagcagctgcctgagaagtacaaagagattttcttcgaccagagcaagaacggctacgccggctacattgacggcggagccagccaggaagagttctacaagttcatcaagcccatcctggaaaagatggacggcaccgaggaactgctcgtgaagctgaacagagaggacctgctgcggaagcagcggaccttcgacaacggcagcatcccccaccagatccacctgggagagctgcacgccattctgcggcggcaggaagatttttacccattcctgaaggacaaccgggaaaagatcgagaagatcctgaccttccgcatcccctactacgtgggccctctggccaggggaaacagcagattcgcctggatgaccagaaagagcgaggaaaccatcaccccctggaacttcgaggaagtggtggacaagggcgcttccgcccagagcttcatcgagcggatgaccaacttcgataagaacctgcccaacgagaaggtgctgcccaagcacagcctgctgtacgagtacttcaccgtgtataacgagctgaccaaagtgaaatacgtgaccgagggaatgagaaagcccgccttcctgagcggcgagcagaaaaaggccatcgtggacctgctgttcaagaccaaccggaaagtgaccgtgaagcagctgaaagaggactacttcaagaaaatcgagtgcttcgactccgtggaaatctccggcgtggaagatcggttcaacgcctccctgggcacataccacgatctgctgaaaattatcaaggacaaggacttcctggacaatgaggaaaacgaggacattctggaagatatcgtgctgaccctgacactgtttgaggacagagagatgatcgaggaacggctgaaaacctatgcccacctgttcgacgacaaagtgatgaagcagctgaagcggcggagatacaccggctggggcaggctgagccggaagctgatcaacggcatccgggacaagcagtccggcaagacaatcctggatttcctgaagtccgacggcttcgccaacagaaacttcatgcagctgatccacgacgacagcctgacctttaaagaggacatccagaaagcccaggtgtccggccagggcgatagcctgcacgagcacattgccaatctggccggcagccccgccattaagaagggcatcctgcagacagtgaaggtggtggacgagctcgtgaaagtgatgggccggcacaagcccgagaacatcgtgatcgaaatggccagagagaaccagaccacccagaagggacagaagaacagccgcgagagaatgaagcggatcgaagagggcatcaaagagctgggcagccagatcctgaaagaacaccccgtggaaaacacccagctgcagaacgagaagctgtacctgtactacctgcagaatgggcgggatatgtacgtggaccaggaactggacatcaaccggctgtccgactacgatgtggaccatatcgtgcctcagagctttctgaaggacgactccatcgacaacaaggtgctgaccagaagcgacaagaaccggggcaagagcgacaacgtgccctccgaagaggtcgtgaagaagatgaagaactactggcggcagctgctgaacgccaagctgattacccagagaaagttcgacaatctgaccaaggccgagagaggcggcctgagcgaactggataaggccggcttcatcaagagacagctggtggaaacccggcagatcacaaagcacgtggcacagatcctggactcccggatgaacactaagtacgacgagaatgacaagctgatccgggaagtgaaagtgatcaccctgaagtccaagctggtgtccgatttccggaaggatttccagttttacaaagtgcgcgagatcaacaactaccaccacgcccacgacgcctacctgaacgccgtcgtgggaaccgccctgatcaaaaagtaccctaagctggaaagcgagttcgtgtacggcgactacaaggtgtacgacgtgcggaagatgatcgccaagagcgagcaggaaatcggcaaggctaccgccaagtacttcttctacagcaacatcatgaactttttcaagaccgagattaccctggccaacggcgagatccggaagcggcctctgatcgagacaaacggcgaaaccggggagatcgtgtgggataagggccgggattttgccaccgtgcggaaagtgctgagcatgccccaagtgaatatcgtgaaaaagaccgaggtgcagacaggcggcttcagcaaagagtctatcctgcccaagaggaacagcgataagctgatcgccagaaagaaggactgggaccctaagaagtacggcggcttcgacagccccaccgtggcctattctgtgctggtggtggccaaagtggaaaagggcaagtccaagaaactgaagagtgtgaaagagctgctggggatcaccatcatggaaagaagcagcttcgagaagaatcccatcgactttctggaagccaagggctacaaagaagtgaaaaaggacctgatcatcaagctgcctaagtactccctgttcgagctggaaaacggccggaagagaatgctggcctctgccggcgaactgcagaagggaaacgaactggccctgccctccaaatatgtgaacttcctgtacctggccagccactatgagaagctgaagggctcccccgaggataatgagcagaaacagctgtttgtggaacagcacaagcactacctggacgagatcatcgagcagatcagcgagttctccaagagagtgatcctggccgacgctaatctggacaaagtgctgtccgcctacaacaagcaccgggataagcccatcagagagcaggccgagaatatcatccacctgtttaccctgaccaatctgggagcccctgccgccttcaagtactttgacaccaccatcgaccggaagaggtacaccagcaccaaagaggtgctggacgccaccctgatccaccagagcatcaccggcctgtacgagacacggatcgacctgtctcagctgggaggcgacaaaaggccggcggccacgaaaaaggccggccaggcaaaaaagaaaaagtgataataggctggagcctcggtggccatgcttcttgccccttgggcctccccccagcccctcctccccttcctgcacccgtacccccgtggtctttgaataaagtctgagtgggcggcaaaaaaaaaaaaaaaaaaaaaaaaaaaaaaagcatatgactaaaaaaaaaaaaaaaaaaaaaaaaaaaaaaaaaaaaaaaaaaaaaaaaaaaaaaaaaaaaaaaaaaaaaa

SEQ ID NO: 2 - DNA, 4555 bp, synthetic construct
  source 1..4555: mol_type = other DNA
gggagacccaagctggctagcgtttaaacttaagcttggtaccgagctcggatccactagtccagtgtggtggaattcgggaaataagagagaaaagaagagtaagaagaaatataagagccaccatggcccctaaaaaaaaaagaaaagttggaatccacggcgtgcccgccgccgacaagaagtactccatcggcctggacatcggcaccaacagcgtgggctgggccgtgatcaccgacgagtacaaggtgcccagcaagaagttcaaggtgctgggcaacaccgaccggcacagcatcaagaagaacctgatcggcgccctgctgttcgacagcggcgagaccgccgaggccacccggctgaagcggaccgcccggcggcggtacacccggcggaagaaccggatctgctacctgcaggagatcttcagcaacgagatggccaaggtggacgacagcttcttccaccggctggaggagagcttcctggtggaggaggacaagaagcacgagcggcaccccatcttcggcaacatcgtggacgaggtggcctaccacgagaagtaccccaccatctaccacctgcggaagaagctggtggacagcaccgacaaggccgacctgcggctgatctacctggccctggcccacatgatcaagttccggggccacttcctgatcgagggcgacctgaaccccgacaacagcgacgtggacaagctgttcatccagctggtgcagacctacaaccagctgttcgaggagaaccccatcaacgccagcggcgtggacgccaaggccatcctgagcgcccggctgagcaagagccggcggctggagaacctgatcgcccagctgcccggcgagaagaagaacggcctgttcggcaacctgatcgccctgagcctgggcctgacccccaacttcaagagcaacttcgacctggccgaggacgccaagctgcagctgagcaaggacacctacgacgacgacctggacaacctgctggcccagatcggcgaccagtacgccgacctgttcctggccgccaagaacctgagcgacgccatcctgctgagcgacatcctgcgggtgaacaccgagatcaccaaggcccccctgagcgccagcatgatcaagcggtacgacgagcaccaccaggacctgaccctgctgaaggccctggtgcggcagcagctgcccgagaagtacaaggagatcttcttcgaccagagcaagaacggctacgccggctacatcgacggcggcgccagccaggaggagttctacaagttcatcaagcccatcctggagaagatggacggcaccgaggagctgctggtgaagctgaaccgggaggacctgctgcggaagcagcggaccttcgacaacggcagcatcccccaccagatccacctgggcgagctgcacgccatcctgcggcggcaggaggacttctaccccttcctgaaggacaaccgggagaagatcgagaagatcctgaccttccggatcccctactacgtgggccccctggcccggggcaacagccggttcgcctggatgacccggaagagcgaggagaccatcaccccctggaacttcgaggaggtggtggacaagggcgccagcgcccagagcttcatcgagcggatgaccaacttcgacaagaacctgcccaacgagaaggtgctgcccaagcacagcctgctgtacgagtacttcaccgtgtacaacgagctgaccgccgtgaagtacgtgaccgagggcatgcggaagcccgccttcctgagcggcgagcagaagaaggccatcgtggacctgctgttcaagaccaaccggaaggtgaccgtgaagcagctgaaggaggactacttcaagaagatcgagtgcttcgacagcgtggagatcagcggcgtggaggaccggttcaacgccagcctgggcacctaccacgacctgctgaagatcatcaaggacaaggacttcctggacaacgaggagaacgaggacatcctggaggacatcgtgctgaccctgaccctgttcgaggaccgggagatgatcgaggagcggctgaagacctacgcccacctgttcgacgacaaggtgatgaagcagctgaagcggcggcggtacaccggctggggccgcctgagccggaagctgatcaacggcatccgggacaagcagagcggcaagaccatcctggacttcctgaagagcgacggcttcgccaacgccaacttcatggccctgatcgccgacgacagcctgaccttcaaggaggacatccagaaggcccaggtgagcggccagggcgacagcctgcacgagcacatcgccaacctggccggcagccccgccatcaagaagggcatcctgcagaccgtgaaggtggtggacgagctggtgaaggtgatgggccggcacaagcccgagaacatcgtgatcgagatggcccgggagaaccagaccacccagaagggccagaagaacagccgggagcggatgaagcggatcgaggagggcatcaaggagctgggcagccagatcctgaaggagcaccccgtggagaacacccagctgcagaacgagaagctgtacctgtactacctgcagaacggccgggacatgtacgtggaccaggagctggacatcaaccggctgagcgactacgacgtggaccacatcgtgccccagagcttcctgaaggacgacagcatcgacaacaaggtgctgacccggagcgacaagaaccggggcaagagcgacaacgtgcccagcgaggaggtggtgaagaagatgaagaactactggcggcagctgctgaacgccaagctgatcacccagcggaagttcgacaacctgaccaaggccgagcggggcggcctgagcgagctggacaaggccggcttcatcaagcggcagctggtggagacccggcagatcaccaagcacgtggcccagatcctggacagccggatgaacaccaagtacgacgagaacgacaagctgatccgggaggtgaaggtgatcaccctgaagagcaagctggtgagcgacttccggaaggacttccagttctacaaggtgcgggagatcaacaactaccaccacgcccacgacgcctacctgaacgccgtggtgggcaccgccctgatcaagaagtaccccaagctggagagcgagttcgtgtacggcgactacaaggtgtacgacgtgcggaagatgatcgccaagagcgagcaggagatcggcaaggccaccgccaagtacttcttctacagcaacatcatgaacttcttcaagaccgagatcaccctggccaacggcgagatccggaagcggcccctgatcgagaccaacggcgagaccggcgagatcgtgtgggacaagggccgggacttcgccaccgtgcggaaggtgctgagcatgccccaggtgaacatcgtgaagaagaccgaggtgcagaccggcggcttcagcaaggagagcatcctgcccaagcggaacagcgacaagctgatcgcccggaagaaggactgggaccccaagaagtacggcggcttcgacagccccaccgtggcctacagcgtgctggtggtggccaaggtggagaagggcaagagcaagaagctgaagagcgtgaaggagctgctgggcatcaccatcatggagcggagcagcttcgagaagaaccccatcgacttcctggaggccaagggctacaaggaggtgaagaaggacctgatcatcaagctgcccaagtacagcctgttcgagctggagaacggccggaagcggatgctggccagcgccggcgagctgcagaagggcaacgagctggccctgcccagcaagtacgtgaacttcctgtacctggccagccactacgagaagctgaagggcagccccgaggacaacgagcagaagcagctgttcgtggagcagcacaagcactacctggacgagatcatcgagcagatcagcgagttcagcaagcgggtgatcctggccgacgccaacctggacaaggtgctgagcgcctacaacaagcaccgggacaagcccatccgggagcaggccgagaacatcatccacctgttcaccctgaccaacctgggcgcccccgccgccttcaagtacttcgacaccaccatcgaccggaagcggtacaccagcaccaaggaggtgctggacgccaccctgatccaccagagcatcaccggcctgtacgagacccggatcgacctgagccagctgggcggcgacaagcggcccgccgccaccaagaaggccggccaggccaagaagaagaagtgataataggctggagcctcggtggccatgcttcttgccccttgggcctccccccagcccctcctccccttcctgcacccgtacccccgtggtctttgaataaagtctgagtgggcggcaaaaaaaaaaaaaaaaaaaaaaaaaaaaaaagcatatgactaaaaaaaaaaaaaaaaaaaaaaaaaaaaaaaaaaaaaaaaaaaaaaaaaaaaaaaaaaaaaaaaaaaaaa

SEQ ID NO: 3 - DNA, 4555 bp, synthetic construct
  source 1..4555: mol_type = other DNA
gggagacccaagctggctagcgtttaaacttaagcttggtaccgagctcggatccactagtccagtgtggtggaattcgggaaataagagagaaaagaagagtaagaagaaatataagagccaccatggcccctaaaaaaaaaagaaaagttggaatccacggcgtgcccgccgccgacaagaagtacagcatcggcctggacatcggcaccaacagcgtgggctgggccgtgatcaccgacgagtacaaggtgcccagcaagaagttcaaggtgctgggcaacaccgaccggcacagcatcaagaagaacctgatcggcgccctgctgttcgacagcggcgagaccgccgaggccacccggctgaagcggaccgcccggcggcggtacacccggcggaagaaccggatctgctacctgcaggagatcttcagcaacgagatggccaaggtggacgacagcttcttccaccggctggaggagagcttcctggtggaggaggacaagaagcacgagcggcaccccatcttcggcaacatcgtggacgaggtggcctaccacgagaagtaccccaccatctaccacctgcggaagaagctggtggacagcaccgacaaggccgacctgcggctgatctacctggccctggcccacatgatcaagttccggggccacttcctgatcgagggcgacctgaaccccgacaacagcgacgtggacaagctgttcatccagctggtgcagacctacaaccagctgttcgaggagaaccccatcaacgccagcggcgtggacgccaaggccatcctgagcgcccggctgagcaagagccggcggctggagaacctgatcgcccagctgcccggcgagaagaagaacggcctgttcggcaacctgatcgccctgagcctgggcctgacccccaacttcaagagcaacttcgacctggccgaggacgccaagctgcagctgagcaaggacacctacgacgacgacctggacaacctgctggcccagatcggcgaccagtacgccgacctgttcctggccgccaagaacctgagcgacgccatcctgctgagcgacatcctgcgggtgaacaccgagatcaccaaggcccccctgagcgccagcatgatcaagcggtacgacgagcaccaccaggacctgaccctgctgaaggccctggtgcggcagcagctgcccgagaagtacaaggagatcttcttcgaccagagcaagaacggctacgccggctacatcgacggcggcgccagccaggaggagttctacaagttcatcaagcccatcctggagaagatggacggcaccgaggagctgctggtgaagctgaaccgggaggacctgctgcggaagcagcggaccttcgacaacggcagcatcccccaccagatccacctgggcgagctgcacgccatcctgcggcggcaggaggacttctaccccttcctgaaggacaaccgggagaagatcgagaagatcctgaccttccggatcccctactacgtgggccccctggcccggggcaacagccggttcgcctggatgacccggaagagcgaggagaccatcaccccctggaacttcgaggaggtggtggacaagggcgccagcgcccagagcttcatcgagcggatgaccgccttcgacaagaacctgcccaacgagaaggtgctgcccaagcacagcctgctgtacgagtacttcaccgtgtacaacgagctgaccaaggtgaagtacgtgaccgagggcatgcggaagcccgccttcctgagcggcgagcagaagaaggccatcgtggacctgctgttcaagaccaaccggaaggtgaccgtgaagcagctgaaggaggactacttcaagaagatcgagtgcttcgacagcgtggagatcagcggcgtggaggaccggttcaacgccagcctgggcacctaccacgacctgctgaagatcatcaaggacaaggacttcctggacaacgaggagaacgaggacatcctggaggacatcgtgctgaccctgaccctgttcgaggaccgggagatgatcgaggagcggctgaagacctacgcccacctgttcgacgacaaggtgatgaagcagctgaagcggcggcggtacaccggctggggcgccctgagccggaagctgatcaacggcatccgggacaagcagagcggcaagaccatcctggacttcctgaagagcgacggcttcgccaaccggaacttcatggccctgatccacgacgacagcctgaccttcaaggaggacatccagaaggcccaggtgagcggccagggcgacagcctgcacgagcacatcgccaacctggccggcagccccgccatcaagaagggcatcctgcagaccgtgaaggtggtggacgagctggtgaaggtgatgggccggcacaagcccgagaacatcgtgatcgagatggcccgggagaaccagaccacccagaagggccagaagaacagccgggagcggatgaagcggatcgaggagggcatcaaggagctgggcagccagatcctgaaggagcaccccgtggagaacacccagctgcagaacgagaagctgtacctgtactacctgcagaacggccgggacatgtacgtggaccaggagctggacatcaaccggctgagcgactacgacgtggaccacatcgtgccccagagcttcctgaaggacgacagcatcgacaacaaggtgctgacccggagcgacaagaaccggggcaagagcgacaacgtgcccagcgaggaggtggtgaagaagatgaagaactactggcggcagctgctgaacgccaagctgatcacccagcggaagttcgacaacctgaccaaggccgagcggggcggcctgagcgagctggacaaggccggcttcatcaagcggcagctggtggagacccgggccatcaccaagcacgtggcccagatcctggacagccggatgaacaccaagtacgacgagaacgacaagctgatccgggaggtgaaggtgatcaccctgaagagcaagctggtgagcgacttccggaaggacttccagttctacaaggtgcgggagatcaacaactaccaccacgcccacgacgcctacctgaacgccgtggtgggcaccgccctgatcaagaagtaccccaagctggagagcgagttcgtgtacggcgactacaaggtgtacgacgtgcgcaagatgatcgccaagagcgagcaggagatcggcaaggccaccgccaagtacttcttctacagcaacatcatgaacttcttcaagaccgagatcaccctggccaacggcgagatccggaagcggcccctgatcgagaccaacggcgagaccggcgagatcgtgtgggacaagggccgggacttcgccaccgtgcggaaggtgctgagcatgccccaggtgaacatcgtgaagaagaccgaggtgcagaccggcggcttcagcaaggagtccatcctgcccaagcggaacagcgacaagctgatcgcccggaagaaggactgggaccccaagaagtacggcggcttcgacagccccaccgtggcctacagcgtgctggtggtggccaaggtggagaagggcaagagcaagaagctgaagagcgtgaaggagctgctgggcatcaccatcatggagcggagcagcttcgagaagaaccccatcgacttcctggaggccaagggctacaaggaggtgaagaaggacctgatcatcaagctgcccaagtacagcctgttcgagctggagaacggccggaagcggatgctggccagcgccggcgagctgcagaagggcaacgagctggccctgcccagcaagtacgtgaacttcctgtacctggccagccactacgagaagctgaagggcagccccgaggacaacgagcagaagcagctgttcgtggagcagcacaagcactacctggacgagatcatcgagcagatcagcgagttcagcaagcgggtgatcctggccgacgccaacctggacaaggtgctgagcgcctacaacaagcaccgggacaagcccatccgggagcaggccgagaacatcatccacctgttcaccctgaccaacctgggcgcccccgccgccttcaagtacttcgacaccaccatcgaccggaagcggtacaccagcaccaaggaggtgctggacgccaccctgatccaccagagcatcaccggcctgtacgagacccggatcgacctgagccagctgggcggcgacaagcggcccgccgccaccaagaaggccggccaggccaagaagaagaagtgataataggctggagcctcggtggccatgcttcttgccccttgggcctccccccagcccctcctccccttcctgcacccgtacccccgtggtctttgaataaagtctgagtgggcggcaaaaaaaaaaaaaaaaaaaaaaaaaaaaaaagcatatgactaaaaaaaaaaaaaaaaaaaaaaaaaaaaaaaaaaaaaaaaaaaaaaaaaaaaaaaaaaaaaaaaaaaaaa

SEQ ID NO: 4 - DNA, 4555 bp, synthetic construct
  source 1..4555: mol_type = other DNA
gggagacccaagctggctagcgtttaaacttaagcttggtaccgagctcggatccactagtccagtgtggtggaattcgggaaataagagagaaaagaagagtaagaagaaatataagagccaccatggccccaaagaagaagcggaaggtcggtatccacggagtcccagcagccgacaagaagtacagcatcggcctggacatcggcaccaactctgtgggctgggccgtgatcaccgacgagtacaaggtgcccagcaagaaattcaaggtgctgggcaacaccgaccggcacagcatcaagaagaacctgatcggagccctgctgttcgacagcggcgaaacagccgaggccacccggctgaagagaaccgccagaagaagatacaccagacggaagaaccggatctgctatctgcaagagatcttcagcaacgagatggccaaggtggacgacagcttcttccacagactggaagagtccttcctggtggaagaggataagaagcacgagcggcaccccatcttcggcaacatcgtggacgaggtggcctaccacgagaagtaccccaccatctaccacctgagaaagaaactggtggacagcaccgacaaggccgacctgcggctgatctatctggccctggcccacatgatcaagttccggggccacttcctgatcgagggcgacctgaaccccgacaacagcgacgtggacaagctgttcatccagctggtgcagacctacaaccagctgttcgaggaaaaccccatcaacgccagcggcgtggacgccaaggccatcctgtctgccagactgagcaagagcagacggctggaaaatctgatcgcccagctgcccggcgagaagaagaatggcctgttcggaaacctgattgccctgagcctgggcctgacccccaacttcaagagcaacttcgacctggccgaggatgccaaactgcagctgagcaaggacacctacgacgacgacctggacaacctgctggcccagatcggcgaccagtacgccgacctgtttctggccgccaagaacctgtccgacgccatcctgctgagcgacatcctgagagtgaacaccgagatcaccaaggcccccctgagcgcctctatgatcaagagatacgacgagcaccaccaggacctgaccctgctgaaagctctcgtgcggcagcagctgcctgagaagtacaaagagattttcttcgaccagagcaagaacggctacgccggctacattgacggcggagccagccaggaagagttctacaagttcatcaagcccatcctggaaaagatggacggcaccgaggaactgctcgtgaagctgaacagagaggacctgctgcggaagcagcggaccttcgacaacggcagcatcccccaccagatccacctgggagagctgcacgccattctgcggcggcaggaagatttttacccattcctgaaggacaaccgggaaaagatcgagaagatcctgaccttccgcatcccctactacgtgggccctctggccaggggaaacagcagattcgcctggatgaccagaaagagcgaggaaaccatcaccccctggaacttcgaggaagtggtggacaagggcgcttccgcccagagcttcatcgagcggatgaccaacttcgataagaacctgcccaacgagaaggtgctgcccaagcacagcctgctgtacgagtacttcaccgtgtataacgagctgaccaaagtgaaatacgtgaccgagggaatgagaaagcccgccttcctgagcggcgagcagaaaaaggccatcgtggacctgctgttcaagaccaaccggaaagtgaccgtgaagcagctgaaagaggactacttcaagaaaatcgagtgcttcgactccgtggaaatctccggcgtggaagatcggttcaacgcctccctgggcacataccacgatctgctgaaaattatcaaggacaaggacttcctggacaatgaggaaaacgaggacattctggaagatatcgtgctgaccctgacactgtttgaggacagagagatgatcgaggaacggctgaaaacctatgcccacctgttcgacgacaaagtgatgaagcagctgaagcggcggagatacaccggctggggcaggctgagccggaagctgatcaacggcatccgggacaagcagtccggcaagacaatcctggatttcctgaagtccgacggcttcgccaacgccaacttcatgcagctgatccacgacgacagcctgacctttaaagaggacatccagaaagcccaggtgtccggccagggcgatagcctgcacgagcacattgccaatctggccggcagccccgccattaagaagggcatcctgcagacagtgaaggtggtggacgagctcgtgaaagtgatgggccggcacaagcccgagaacatcgtgatcgaaatggccagagagaaccagaccacccagaagggacagaagaacagccgcgagagaatgaagcggatcgaagagggcatcaaagagctgggcagccagatcctgaaagaacaccccgtggaaaacacccagctgcagaacgagaagctgtacctgtactacctgcagaatgggcgggatatgtacgtggaccaggaactggacatcaaccggctgtccgactacgatgtggaccatatcgtgcctcagagctttctgaaggacgactccatcgacaacaaggtgctgaccagaagcgacaagaaccggggcaagagcgacaacgtgccctccgaagaggtcgtgaagaagatgaagaactactggcggcagctgctgaacgccaagctgattacccagagaaagttcgacaatctgaccaaggccgagagaggcggcctgagcgaactggataaggccggcttcatcaagagacagctggtggaaacccggcagatcacaaagcacgtggcacagatcctggactcccggatgaacactaagtacgacgagaatgacaagctgatccgggaagtgaaagtgatcaccctgaagtccaagctggtgtccgatttccggaaggatttccagttttacaaagtgcgcgagatcaacaactaccaccacgcccacgacgcctacctgaacgccgtcgtgggaaccgccctgatcaaaaagtaccctaagctggaaagcgagttcgtgtacggcgactacaaggtgtacgacgtgcggaagatgatcgccaagagcgagcaggaaatcggcaaggctaccgccaagtacttcttctacagcaacatcatgaactttttcaagaccgagattaccctggccaacggcgagatccggaagcggcctctgatcgagacaaacggcgaaaccggggagatcgtgtgggataagggccgggattttgccaccgtgcggaaagtgctgagcatgccccaagtgaatatcgtgaaaaagaccgaggtgcagacaggcggcttcagcaaagagtctatcctgcccaagaggaacagcgataagctgatcgccagaaagaaggactgggaccctaagaagtacggcggcttcgacagccccaccgtggcctattctgtgctggtggtggccaaagtggaaaagggcaagtccaagaaactgaagagtgtgaaagagctgctggggatcaccatcatggaaagaagcagcttcgagaagaatcccatcgactttctggaagccaagggctacaaagaagtgaaaaaggacctgatcatcaagctgcctaagtactccctgttcgagctggaaaacggccggaagagaatgctggcctctgccggcgaactgcagaagggaaacgaactggccctgccctccaaatatgtgaacttcctgtacctggccagccactatgagaagctgaagggctcccccgaggataatgagcagaaacagctgtttgtggaacagcacaagcactacctggacgagatcatcgagcagatcagcgagttctccaagagagtgatcctggccgacgctaatctggacaaagtgctgtccgcctacaacaagcaccgggataagcccatcagagagcaggccgagaatatcatccacctgtttaccctgaccaatctgggagcccctgccgccttcaagtactttgacaccaccatcgaccggaagaggtacaccagcaccaaagaggtgctggacgccaccctgatccaccagagcatcaccggcctgtacgagacacggatcgacctgtctcagctgggaggcgacaaaaggccggcggccacgaaaaaggccggccaggcaaaaaagaaaaagtgataataggctggagcctcggtggccatgcttcttgccccttgggcctccccccagcccctcctccccttcctgcacccgtacccccgtggtctttgaataaagtctgagtgggcggcaaaaaaaaaaaaaaaaaaaaaaaaaaaaaaagcatatgactaaaaaaaaaaaaaaaaaaaaaaaaaaaaaaaaaaaaaaaaaaaaaaaaaaaaaaaaaaaaaaaaaaaaaa

SEQ ID NO: 5 - DNA, 5170 bp, synthetic construct
  source 1..5170: mol_type = other DNA
gggagacccaagctggctagcgtttaaacttaagcttggtaccgagctcggatccactagtccagtgtggtggaattcgggaaataagagagaaaagaagagtaagaagaaatataagagccaccatgaagagaacagctgatggaagtgaatttgagtcccccaagaagaagcggaaggtgagcgaggtggagttcagccacgagtactggatgcggcacgccctgaccctggccaagcgggcccgggacgagcgggaggtgcccgtgggcgccgtgctggtgctgaacaaccgggtgatcggcgagggctggaaccgggccatcggcctgcacgaccccaccgcccacgccgagatcatggccctgcggcagggcggcctggtgatgcagaactaccggctgatcgacgccaccctgtacgtgaccttcgagccctgcgtgatgtgcgccggcgccatgatccacagccggatcggccgggtggtgttcggcgtgcggaacagcaagcggggcgccgccggcagcctgatgaacgtgctgaactaccccggcatgaaccaccgggtggagatcaccgagggcatcctggccgacgagtgcgccgccctgctgtgcgacttctaccggatgccccggcaggtgttcaacgcccagaagaaggcccagagcagcatcaacagcggcggcagcagcggcggcagcagcggcagcgagacccccggcacctccgagagcgccacccccgagagctccggcggcagcagcggcggcagcgacaagaagtacagcatcggcctggccatcggcaccaacagcgtgggctgggccgtgatcaccgacgagtacaaggtgcccagcaagaagttcaaggtgctgggcaacaccgaccggcacagcatcaagaagaacctgatcggcgccctgctgttcgacagcggcgagaccgccgaggccacccggctgaagcggaccgcccggcggcggtacacccggcggaagaaccggatctgctacctgcaggagatcttcagcaacgagatggccaaggtggacgacagcttcttccaccggctggaggagagcttcctggtggaggaggacaagaagcacgagcggcaccccatcttcggcaacatcgtggacgaggtggcctaccacgagaagtaccccaccatctaccacctgcggaagaagctggtggacagcaccgacaaggccgacctgcggctgatctacctggccctggcccacatgatcaagttccggggccacttcctgatcgagggcgacctgaaccccgacaacagcgacgtggacaagctgttcatccagctggtgcagacctacaaccagctgttcgaggagaaccccatcaacgccagcggcgtggacgccaaggccatcctgagcgcccggctgagcaagagccggcggctggagaacctgatcgcccagctgcccggcgagaagaagaacggcctgttcggcaacctgatcgccctgagcctgggcctgacccccaacttcaagagcaacttcgacctggccgaggacgccaagctgcagctgagcaaggacacctacgacgacgacctggacaacctgctggcccagatcggcgaccagtacgccgacctgttcctggccgccaagaacctgagcgacgccatcctgctgagcgacatcctgcgggtgaacaccgagatcaccaaggcccccctgagcgccagcatgatcaagcggtacgacgagcaccaccaggacctgaccctgctgaaggccctggtgcggcagcagctgcccgagaagtacaaggagatcttcttcgaccagagcaagaacggctacgccggctacatcgacggcggcgccagccaggaggagttctacaagttcatcaagcccatcctggagaagatggacggcaccgaggagctgctggtgaagctgaaccgggaggacctgctgcggaagcagcggaccttcgacaacggcagcatcccccaccagatccacctgggcgagctgcacgccatcctgcggcggcaggaggacttctaccccttcctgaaggacaaccgggagaagatcgagaagatcctgaccttccggatcccctactacgtgggccccctggcccggggcaacagccggttcgcctggatgacccggaagagcgaggagaccatcaccccctggaacttcgaggaggtggtggacaagggcgccagcgcccagagcttcatcgagcggatgaccaacttcgacaagaacctgcccaacgagaaggtgctgcccaagcacagcctgctgtacgagtacttcaccgtgtacaacgagctgaccaaggtgaagtacgtgaccgagggcatgcggaagcccgccttcctgagcggcgagcagaagaaggccatcgtggacctgctgttcaagaccaaccggaaggtgaccgtgaagcagctgaaggaggactacttcaagaagatcgagtgcttcgacagcgtggagatcagcggcgtggaggaccggttcaacgccagcctgggcacctaccacgacctgctgaagatcatcaaggacaaggacttcctggacaacgaggagaacgaggacatcctggaggacatcgtgctgaccctgaccctgttcgaggaccgggagatgatcgaggagcggctgaagacctacgcccacctgttcgacgacaaggtgatgaagcagctgaagcggcggcggtacaccggctggggccggctgagccggaagctgatcaacggcatccgggacaagcagagcggcaagaccatcctggacttcctgaagagcgacggcttcgccaaccggaacttcatgcagctgatccacgacgacagcctgaccttcaaggaggacatccagaaggcccaggtgagcggccagggcgacagcctgcacgagcacatcgccaacctggccggcagccccgccatcaagaagggcatcctgcagaccgtgaaggtggtggacgagctggtgaaggtgatgggccggcacaagcccgagaacatcgtgatcgagatggcccgggagaaccagaccacccagaagggccagaagaacagccgggagcggatgaagcggatcgaggagggcatcaaggagctgggcagccagatcctgaaggagcaccccgtggagaacacccagctgcagaacgagaagctgtacctgtactacctgcagaacggccgggacatgtacgtggaccaggagctggacatcaaccggctgagcgactacgacgtggaccacatcgtgccccagagcttcctgaaggacgacagcatcgacaacaaggtgctgacccggagcgacaagaaccggggcaagagcgacaacgtgcccagcgaggaggtggtgaagaagatgaagaactactggcggcagctgctgaacgccaagctgatcacccagcggaagttcgacaacctgaccaaggccgagcggggcggcctgagcgagctggacaaggccggcttcatcaagcggcagctggtggagacccggcagatcaccaagcacgtggcccagatcctggacagccggatgaacaccaagtacgacgagaacgacaagctgatccgggaggtgaaggtgatcaccctgaagagcaagctggtgagcgacttccggaaggacttccagttctacaaggtgcgggagatcaacaactaccaccacgcccacgacgcctacctgaacgccgtggtgggcaccgccctgatcaagaagtaccccaagctggagagcgagttcgtgtacggcgactacaaggtgtacgacgtgcggaagatgatcgccaagagcgagcaggagatcggcaaggccaccgccaagtacttcttctacagcaacatcatgaacttcttcaagaccgagatcaccctggccaacggcgagatccggaagcggcccctgatcgagaccaacggcgagaccggcgagatcgtgtgggacaagggccgggacttcgccaccgtgcggaaggtgctgagcatgccccaggtgaacatcgtgaagaagaccgaggtgcagaccggcggcttcagcaaggagagcatcctgcccaagcggaacagcgacaagctgatcgcccggaagaaggactgggaccccaagaagtacggcggcttcgacagccccaccgtggcctacagcgtgctggtggtggccaaggtggagaagggcaagagcaagaagctgaagagcgtgaaggagctgctgggcatcaccatcatggagcggagcagcttcgagaagaaccccatcgacttcctggaggccaagggctacaaggaggtgaagaaggacctgatcatcaagctgcccaagtacagcctgttcgagctggagaacggccggaagcggatgctggccagcgccggcgagctgcagaagggcaacgagctggccctgcccagcaagtacgtgaacttcctgtacctggccagccactacgagaagctgaagggcagccccgaggacaacgagcagaagcagctgttcgtggagcagcacaagcactacctggacgagatcatcgagcagatcagcgagttcagcaagcgggtgatcctggccgacgccaacctggacaaggtgctgagcgcctacaacaagcaccgggacaagcccatccgggagcaggccgagaacatcatccacctgttcaccctgaccaacctgggcgcccccgccgccttcaagtacttcgacaccaccatcgaccggaagcggtacaccagcaccaaggaggtgctggacgccaccctgatccaccagagcatcaccggcctgtacgagacccggatcgacctgagccagctgggcggcgacagcggcggcagcaagcggaccgccgacggcagcgagttcgagcccaagaagaagcggaaggtgtgataataggctggagcctcggtggccatgcttcttgccccttgggcctccccccagcccctcctccccttcctgcacccgtacccccgtggtctttgaataaagtctgagtgggcggcaaaaaaaaaaaaaaaaaaaaaaaaaaaaaaagcatatgactaaaaaaaaaaaaaaaaaaaaaaaaaaaaaaaaaaaaaaaaaaaaaaaaaaaaaaaaaaaaaaaaaaaaaa

SEQ ID NO: 6 - DNA, 5170 bp, synthetic construct
  source 1..5170: mol_type = other DNA
gggagacccaagctggctagcgtttaaacttaagcttggtaccgagctcggatccactagtccagtgtggtggaattcgggaaataagagagaaaagaagagtaagaagaaatataagagccaccatgaagagaacagctgatggaagtgaatttgagtcccccaagaagaagcggaaggtgagcgaggtggagttcagccacgagtactggatgcggcacgccctgaccctggccaagcgggcccgggacgagcgggaggtgcccgtgggcgccgtgctggtgctgaacaaccgggtgatcggcgagggctggaaccgggccatcggcctgcacgaccccaccgcccacgccgagatcatggccctgcggcagggcggcctggtgatgcagaactaccggctgatcgacgccaccctgtacgtgaccttcgagccctgcgtgatgtgcgccggcgccatgatccacagccggatcggccgggtggtgttcggcgtgcggaacagcaagcggggcgccgccggcagcctgatgaacgtgctgaactaccccggcatgaaccaccgggtggagatcaccgagggcatcctggccgacgagtgcgccgccctgctgtgcgacttctaccggatgccccggcaggtgttcaacgcccagaagaaggcccagagcagcatcaacagcggcggcagcagcggcggcagcagcggcagcgagacccccggcacctccgagagcgccacccccgagagctccggcggcagcagcggcggcagcgacaagaagtacagcatcggcctggccatcggcaccaacagcgtgggctgggccgtgatcaccgacgagtacaaggtgcccagcaagaagttcaaggtgctgggcaacaccgaccggcacagcatcaagaagaacctgatcggcgccctgctgttcgacagcggcgagaccgccgaggccacccggctgaagcggaccgcccggcggcggtacacccggcggaagaaccggatctgctacctgcaggagatcttcagcaacgagatggccaaggtggacgacagcttcttccaccggctggaggagagcttcctggtggaggaggacaagaagcacgagcggcaccccatcttcggcaacatcgtggacgaggtggcctaccacgagaagtaccccaccatctaccacctgcggaagaagctggtggacagcaccgacaaggccgacctgcggctgatctacctggccctggcccacatgatcaagttccggggccacttcctgatcgagggcgacctgaaccccgacaacagcgacgtggacaagctgttcatccagctggtgcagacctacaaccagctgttcgaggagaaccccatcaacgccagcggcgtggacgccaaggccatcctgagcgcccggctgagcaagagccggcggctggagaacctgatcgcccagctgcccggcgagaagaagaacggcctgttcggcaacctgatcgccctgagcctgggcctgacccccaacttcaagagcaacttcgacctggccgaggacgccaagctgcagctgagcaaggacacctacgacgacgacctggacaacctgctggcccagatcggcgaccagtacgccgacctgttcctggccgccaagaacctgagcgacgccatcctgctgagcgacatcctgcgggtgaacaccgagatcaccaaggcccccctgagcgccagcatgatcaagcggtacgacgagcaccaccaggacctgaccctgctgaaggccctggtgcggcagcagctgcccgagaagtacaaggagatcttcttcgaccagagcaagaacggctacgccggctacatcgacggcggcgccagccaggaggagttctacaagttcatcaagcccatcctggagaagatggacggcaccgaggagctgctggtgaagctgaaccgggaggacctgctgcggaagcagcggaccttcgacaacggcagcatcccccaccagatccacctgggcgagctgcacgccatcctgcggcggcaggaggacttctaccccttcctgaaggacaaccgggagaagatcgagaagatcctgaccttccggatcccctactacgtgggccccctggcccggggcaacagccggttcgcctggatgacccggaagagcgaggagaccatcaccccctggaacttcgaggaggtggtggacaagggcgccagcgcccagagcttcatcgagcggatgaccaacttcgacaagaacctgcccaacgagaaggtgctgcccaagcacagcctgctgtacgagtacttcaccgtgtacaacgagctgaccgccgtgaagtacgtgaccgagggcatgcggaagcccgccttcctgagcggcgagcagaagaaggccatcgtggacctgctgttcaagaccaaccggaaggtgaccgtgaagcagctgaaggaggactacttcaagaagatcgagtgcttcgacagcgtggagatcagcggcgtggaggaccggttcaacgccagcctgggcacctaccacgacctgctgaagatcatcaaggacaaggacttcctggacaacgaggagaacgaggacatcctggaggacatcgtgctgaccctgaccctgttcgaggaccgggagatgatcgaggagcggctgaagacctacgcccacctgttcgacgacaaggtgatgaagcagctgaagcggcggcggtacaccggctggggccggctgagccggaagctgatcaacggcatccgggacaagcagagcggcaagaccatcctggacttcctgaagagcgacggcttcgccaacgccaacttcatggccctgatcgccgacgacagcctgaccttcaaggaggacatccagaaggcccaggtgagcggccagggcgacagcctgcacgagcacatcgccaacctggccggcagccccgccatcaagaagggcatcctgcagaccgtgaaggtggtggacgagctggtgaaggtgatgggccggcacaagcccgagaacatcgtgatcgagatggcccgggagaaccagaccacccagaagggccagaagaacagccgggagcggatgaagcggatcgaggagggcatcaaggagctgggcagccagatcctgaaggagcaccccgtggagaacacccagctgcagaacgagaagctgtacctgtactacctgcagaacggccgggacatgtacgtggaccaggagctggacatcaaccggctgagcgactacgacgtggaccacatcgtgccccagagcttcctgaaggacgacagcatcgacaacaaggtgctgacccggagcgacaagaaccggggcaagagcgacaacgtgcccagcgaggaggtggtgaagaagatgaagaactactggcggcagctgctgaacgccaagctgatcacccagcggaagttcgacaacctgaccaaggccgagcggggcggcctgagcgagctggacaaggccggcttcatcaagcggcagctggtggagacccggcagatcaccaagcacgtggcccagatcctggacagccggatgaacaccaagtacgacgagaacgacaagctgatccgggaggtgaaggtgatcaccctgaagagcaagctggtgagcgacttccggaaggacttccagttctacaaggtgcgggagatcaacaactaccaccacgcccacgacgcctacctgaacgccgtggtgggcaccgccctgatcaagaagtaccccaagctggagagcgagttcgtgtacggcgactacaaggtgtacgacgtgcggaagatgatcgccaagagcgagcaggagatcggcaaggccaccgccaagtacttcttctacagcaacatcatgaacttcttcaagaccgagatcaccctggccaacggcgagatccggaagcggcccctgatcgagaccaacggcgagaccggcgagatcgtgtgggacaagggccgggacttcgccaccgtgcggaaggtgctgagcatgccccaggtgaacatcgtgaagaagaccgaggtgcagaccggcggcttcagcaaggagagcatcctgcccaagcggaacagcgacaagctgatcgcccggaagaaggactgggaccccaagaagtacggcggcttcgacagccccaccgtggcctacagcgtgctggtggtggccaaggtggagaagggcaagagcaagaagctgaagagcgtgaaggagctgctgggcatcaccatcatggagcggagcagcttcgagaagaaccccatcgacttcctggaggccaagggctacaaggaggtgaagaaggacctgatcatcaagctgcccaagtacagcctgttcgagctggagaacggccggaagcggatgctggccagcgccggcgagctgcagaagggcaacgagctggccctgcccagcaagtacgtgaacttcctgtacctggccagccactacgagaagctgaagggcagccccgaggacaacgagcagaagcagctgttcgtggagcagcacaagcactacctggacgagatcatcgagcagatcagcgagttcagcaagcgggtgatcctggccgacgccaacctggacaaggtgctgagcgcctacaacaagcaccgggacaagcccatccgggagcaggccgagaacatcatccacctgttcaccctgaccaacctgggcgcccccgccgccttcaagtacttcgacaccaccatcgaccggaagcggtacaccagcaccaaggaggtgctggacgccaccctgatccaccagagcatcaccggcctgtacgagacccggatcgacctgagccagctgggcggcgacagcggcggcagcaagcggaccgccgacggcagcgagttcgagcccaagaagaagcggaaggtgtgataataggctggagcctcggtggccatgcttcttgccccttgggcctccccccagcccctcctccccttcctgcacccgtacccccgtggtctttgaataaagtctgagtgggcggcaaaaaaaaaaaaaaaaaaaaaaaaaaaaaaagcatatgactaaaaaaaaaaaaaaaaaaaaaaaaaaaaaaaaaaaaaaaaaaaaaaaaaaaaaaaaaaaaaaaaaaaaaa

SEQ ID NO: 7 - DNA, 6610 bp, synthetic construct
  source 1..6610: mol_type = other DNA
gggagacccaagctggctagcgtttaaacttaagcttggtaccgagctcggatccactagtccagtgtggtggaattcgggaaataagagagaaaagaagagtaagaagaaatataagagccaccatgaatcatgatcaagaattcgatcctccaaaggtttatcctcctgttccagctgaaaagagaaagcctattagagttctttctttgttcgacggcatcgccaccggcctgctggtgctgaaggacctgggcatccaggtggaccggtacatcgccagcgaggtgtgcgaggacagcatcaccgtgggcatggtgcggcaccagggcaagatcatgtacgtgggcgacgtgcggagcgtgacccagaagcacatccaggagtggggccccttcgacctggtgatcggcggcagcccctgcaacgacctgagcatcgtgaaccccgcccggaagggcctgtacgagggcaccggccggctgttcttcgagttctaccggctgctgcacgacgcccggcccaaggagggcgacgaccggcccttcttctggctgttcgagaacgtggtggccatgggcgtgagcgacaagcgggacatcagccgcttcctggagagcaaccccgtgatgatcgacgccaaggaggtgagcgccgcccaccgggcccgctacttctggggcaacctgcccggcatgaaccggcccctggccagcaccgtgaacgacaagctggagctgcaggagtgcctggagcacggccggatcgccaagttctccaaggtgcggaccatcaccacccggagcaacagcatcaagcagggcaaggaccagcacttccccgtgttcatgaacgagaaggaggacatcctgtggtgcaccgagatggagcgggtgttcggcttccccgtgcactacaccgacgtgagcaacatgagccggctggcccggcagcggctgctgggccggagctggagcgtgcccgtgatccggcacctgttcgcccccctgaaggagtacttcgcctgcgtgagcagcggcaacagcaacgccaacagccggggccccagcttcagcagcggcctggtgcccctgagcctgcggggcagccacatgggccccatggagatctacaagaccgtgagcgcctggaagcggcagcccgtgcgggtgctgagcctgttccggaacatcgacaaggtgctgaagagcctgggcttcctggagagcggcagcggcagcggcggcggcaccctgaagtacgtggaggacgtgaccaacgtggtgcggcgggacgtggagaagtggggccccttcgacctggtgtacggcagcacccagcccctgggcagcagctgcgaccggtgccccggctggtacatgttccagttccaccggatcctgcagtacgccctgccccggcaggagagccagcggcccttcttctggatcttcatggacaacctgctgctgaccgaggacgaccaggagaccaccacccggttcctgcagaccgaggccgtgaccctgcaggacgtgcggggccgggactaccagaacgccatgcgggtgtggagcaacatccccggcctgaagagcaagcacgcccccctgacccccaaggaggaggagtacctgcaggcccaggtgcggagccggagcaagctggacgcccccaaggtggacctgctggtgaagaactgcctgctgcccctgcgggagtacttcaagtacttcagccagaacagcctgcccctgggcggccccagcagcggcgcccccccccccagcggcggcagccccgccggcagccccaccagcaccgaggagggcaccagcgagagcgccacccccgagagcggccccggcaccagcaccgagcccagcgagggcagcgcccccggcagccccgccggcagccccaccagcaccgaggagggcaccagcaccgagcccagcgagggcagcgcccccggcaccagcaccgagcccagcgagatggacaagaagtacagcatcggcctggccatcggcaccaacagcgtgggctgggccgtgatcaccgacgagtacaaggtgcccagcaagaagttcaaggtgctgggcaacaccgaccggcacagcatcaagaagaacctgatcggcgccctgctgttcgacagcggcgagaccgccgaggccacccggctgaagcggaccgcccggcggcggtacacccggcggaagaaccggatctgctacctgcaggagatcttcagcaacgagatggccaaggtggacgacagcttcttccaccggctggaggagagcttcctggtggaggaggacaagaagcacgagcggcaccccatcttcggcaacatcgtggacgaggtggcctaccacgagaagtaccccaccatctaccacctgcggaagaagctggtggacagcaccgacaaggccgacctgcggctgatctacctggccctggcccacatgatcaagttccggggccacttcctgatcgagggcgacctgaaccccgacaacagcgacgtggacaagctgttcatccagctggtgcagacctacaaccagctgttcgaggagaaccccatcaacgccagcggcgtggacgccaaggccatcctgagcgcccggctgagcaagagccggcggctggagaacctgatcgcccagctgcccggcgagaagaagaacggcctgttcggcaacctgatcgccctgagcctgggcctgacccccaacttcaagagcaacttcgacctggccgaggacgccaagctgcagctgagcaaggacacctacgacgacgacctggacaacctgctggcccagatcggcgaccagtacgccgacctgttcctggccgccaagaacctgagcgacgccatcctgctgagcgacatcctgcgggtgaacaccgagatcaccaaggcccccctgagcgccagcatgatcaagcggtacgacgagcaccaccaggacctgaccctgctgaaggccctggtgcggcagcagctgcccgagaagtacaaggagatcttcttcgaccagagcaagaacggctacgccggctacatcgacggcggcgccagccaggaggagttctacaagttcatcaagcccatcctggagaagatggacggcaccgaggagctgctggtgaagctgaaccgggaggacctgctgcggaagcagcggaccttcgacaacggcagcatcccccaccagatccacctgggcgagctgcacgccatcctgcggcggcaggaggacttctaccccttcctgaaggacaaccgggagaagatcgagaagatcctgaccttccggatcccctactacgtgggccccctggcccggggcaacagccggttcgcctggatgacccggaagagcgaggagaccatcaccccctggaacttcgaggaggtggtggacaagggcgccagcgcccagagcttcatcgagcggatgaccaacttcgacaagaacctgcccaacgagaaggtgctgcccaagcacagcctgctgtacgagtacttcaccgtgtacaacgagctgaccaaggtgaagtacgtgaccgagggcatgcggaagcccgccttcctgagcggcgagcagaagaaggccatcgtggacctgctgttcaagaccaaccggaaggtgaccgtgaagcagctgaaggaggactacttcaagaagatcgagtgcttcgacagcgtggagatcagcggcgtggaggaccggttcaacgccagcctgggcacctaccacgacctgctgaagatcatcaaggacaaggacttcctggacaacgaggagaacgaggacatcctggaggacatcgtgctgaccctgaccctgttcgaggaccgggagatgatcgaggagcggctgaagacctacgcccacctgttcgacgacaaggtgatgaagcagctgaagcggcggcggtacaccggctggggccggctgagccggaagctgatcaacggcatccgggacaagcagagcggcaagaccatcctggacttcctgaagagcgacggcttcgccaaccggaacttcatgcagctgatccacgacgacagcctgaccttcaaggaggacatccagaaggcccaggtgagcggccagggcgacagcctgcacgagcacatcgccaacctggccggcagccccgccatcaagaagggcatcctgcagaccgtgaaggtggtggacgagctggtgaaggtgatgggccggcacaagcccgagaacatcgtgatcgagatggcccgggagaaccagaccacccagaagggccagaagaacagccgggagcggatgaagcggatcgaggagggcatcaaggagctgggcagccagatcctgaaggagcaccccgtggagaacacccagctgcagaacgagaagctgtacctgtactacctgcagaacggccgggacatgtacgtggaccaggagctggacatcaaccggctgagcgactacgacgtggacgccatcgtgccccagagcttcctgaaggacgacagcatcgacaacaaggtgctgacccggagcgacaagaaccggggcaagagcgacaacgtgcccagcgaggaggtggtgaagaagatgaagaactactggcggcagctgctgaacgccaagctgatcacccagcggaagttcgacaacctgaccaaggccgagcggggcggcctgagcgagctggacaaggccggcttcatcaagcggcagctggtggagacccggcagatcaccaagcacgtggcccagatcctggacagccggatgaacaccaagtacgacgagaacgacaagctgatccgggaggtgaaggtgatcaccctgaagagcaagctggtgagcgacttccggaaggacttccagttctacaaggtgcgggagatcaacaactaccaccacgcccacgacgcctacctgaacgccgtggtgggcaccgccctgatcaagaagtaccccaagctggagagcgagttcgtgtacggcgactacaaggtgtacgacgtgcggaagatgatcgccaagagcgagcaggagatcggcaaggccaccgccaagtacttcttctacagcaacatcatgaacttcttcaagaccgagatcaccctggccaacggcgagatccggaagcggcccctgatcgagaccaacggcgagaccggcgagatcgtgtgggacaagggccgggacttcgccaccgtgcggaaggtgctgagcatgccccaggtgaacatcgtgaagaagaccgaggtgcagaccggcggcttcagcaaggagagcatcctgcccaagcggaacagcgacaagctgatcgcccggaagaaggactgggaccccaagaagtacggcggcttcgacagccccaccgtggcctacagcgtgctggtggtggccaaggtggagaagggcaagagcaagaagctgaagagcgtgaaggagctgctgggcatcaccatcatggagcggagcagcttcgagaagaaccccatcgacttcctggaggccaagggctacaaggaggtgaagaaggacctgatcatcaagctgcccaagtacagcctgttcgagctggagaacggccggaagcggatgctggccagcgccggcgagctgcagaagggcaacgagctggccctgcccagcaagtacgtgaacttcctgtacctggccagccactacgagaagctgaagggcagccccgaggacaacgagcagaagcagctgttcgtggagcagcacaagcactacctggacgagatcatcgagcagatcagcgagttcagcaagcgggtgatcctggccgacgccaacctggacaaggtgctgagcgcctacaacaagcaccgggacaagcccatccgggagcaggccgagaacatcatccacctgttcaccctgaccaacctgggcgcccccgccgccttcaagtacttcgacaccaccatcgaccggaagcggtacaccagcaccaaggaggtgctggacgccaccctgatccaccagagcatcaccggcctgtacgagacccggatcgacctgagccagctgggcggcgaccccaagaagaagcggaaggtggaggaccccaagaagaagcggaaggtgggcggcggcggcggcatggacgccaagagcctgaccgcctggagccggaccctggtgaccttcaaggacgtgttcgtggacttcacccgggaggagtggaagctgctggacaccgcccagcagatcgtgtaccggaacgtgatgctggagaactacaagaacctggtgagcctgggctaccagctgaccaagcccgacgtgatcctgcggctggagaagggcgaggagccctgataataggctggagcctcggtggccatgcttcttgccccttgggcctccccccagcccctcctccccttcctgcacccgtacccccgtggtctttgaataaagtctgagtgggcggcaaaaaaaaaaaaaaaaaaaaaaaaaaaaaaagcatatgactaaaaaaaaaaaaaaaaaaaaaaaaaaaaaaaaaaaaaaaaaaaaaaaaaaaaaaaaaaaaaaaaaaaaaa

SEQ ID NO: 8 - DNA, 6610 bp, synthetic construct
  source 1..6610: mol_type = other DNA
gggagacccaagctggctagcgtttaaacttaagcttggtaccgagctcggatccactagtccagtgtggtggaattcgggaaataagagagaaaagaagagtaagaagaaatataagagccaccatgaatcatgatcaagaattcgatcctccaaaggtttatcctcctgttccagctgaaaagagaaagcctattagagttctttctttgttcgacggcatcgccaccggcctgctggtgctgaaggacctgggcatccaggtggaccggtacatcgccagcgaggtgtgcgaggacagcatcaccgtgggcatggtgcggcaccagggcaagatcatgtacgtgggcgacgtgcggagcgtgacccagaagcacatccaggagtggggccccttcgacctggtgatcggcggcagcccctgcaacgacctgagcatcgtgaaccccgcccggaagggcctgtacgagggcaccggccggctgttcttcgagttctaccggctgctgcacgacgcccggcccaaggagggcgacgaccggcccttcttctggctgttcgagaacgtggtggccatgggcgtgagcgacaagcgggacatcagccgcttcctggagagcaaccccgtgatgatcgacgccaaggaggtgagcgccgcccaccgggcccgctacttctggggcaacctgcccggcatgaaccggcccctggccagcaccgtgaacgacaagctggagctgcaggagtgcctggagcacggccggatcgccaagttctccaaggtgcggaccatcaccacccggagcaacagcatcaagcagggcaaggaccagcacttccccgtgttcatgaacgagaaggaggacatcctgtggtgcaccgagatggagcgggtgttcggcttccccgtgcactacaccgacgtgagcaacatgagccggctggcccggcagcggctgctgggccggagctggagcgtgcccgtgatccggcacctgttcgcccccctgaaggagtacttcgcctgcgtgagcagcggcaacagcaacgccaacagccggggccccagcttcagcagcggcctggtgcccctgagcctgcggggcagccacatgggccccatggagatctacaagaccgtgagcgcctggaagcggcagcccgtgcgggtgctgagcctgttccggaacatcgacaaggtgctgaagagcctgggcttcctggagagcggcagcggcagcggcggcggcaccctgaagtacgtggaggacgtgaccaacgtggtgcggcgggacgtggagaagtggggccccttcgacctggtgtacggcagcacccagcccctgggcagcagctgcgaccggtgccccggctggtacatgttccagttccaccggatcctgcagtacgccctgccccggcaggagagccagcggcccttcttctggatcttcatggacaacctgctgctgaccgaggacgaccaggagaccaccacccggttcctgcagaccgaggccgtgaccctgcaggacgtgcggggccgggactaccagaacgccatgcgggtgtggagcaacatccccggcctgaagagcaagcacgcccccctgacccccaaggaggaggagtacctgcaggcccaggtgcggagccggagcaagctggacgcccccaaggtggacctgctggtgaagaactgcctgctgcccctgcgggagtacttcaagtacttcagccagaacagcctgcccctgggcggccccagcagcggcgcccccccccccagcggcggcagccccgccggcagccccaccagcaccgaggagggcaccagcgagagcgccacccccgagagcggccccggcaccagcaccgagcccagcgagggcagcgcccccggcagccccgccggcagccccaccagcaccgaggagggcaccagcaccgagcccagcgagggcagcgcccccggcaccagcaccgagcccagcgagatggacaagaagtacagcatcggcctggccatcggcaccaacagcgtgggctgggccgtgatcaccgacgagtacaaggtgcccagcaagaagttcaaggtgctgggcaacaccgaccggcacagcatcaagaagaacctgatcggcgccctgctgttcgacagcggcgagaccgccgaggccacccggctgaagcggaccgcccggcggcggtacacccggcggaagaaccggatctgctacctgcaggagatcttcagcaacgagatggccaaggtggacgacagcttcttccaccggctggaggagagcttcctggtggaggaggacaagaagcacgagcggcaccccatcttcggcaacatcgtggacgaggtggcctaccacgagaagtaccccaccatctaccacctgcggaagaagctggtggacagcaccgacaaggccgacctgcggctgatctacctggccctggcccacatgatcaagttccggggccacttcctgatcgagggcgacctgaaccccgacaacagcgacgtggacaagctgttcatccagctggtgcagacctacaaccagctgttcgaggagaaccccatcaacgccagcggcgtggacgccaaggccatcctgagcgcccggctgagcaagagccggcggctggagaacctgatcgcccagctgcccggcgagaagaagaacggcctgttcggcaacctgatcgccctgagcctgggcctgacccccaacttcaagagcaacttcgacctggccgaggacgccaagctgcagctgagcaaggacacctacgacgacgacctggacaacctgctggcccagatcggcgaccagtacgccgacctgttcctggccgccaagaacctgagcgacgccatcctgctgagcgacatcctgcgggtgaacaccgagatcaccaaggcccccctgagcgccagcatgatcaagcggtacgacgagcaccaccaggacctgaccctgctgaaggccctggtgcggcagcagctgcccgagaagtacaaggagatcttcttcgaccagagcaagaacggctacgccggctacatcgacggcggcgccagccaggaggagttctacaagttcatcaagcccatcctggagaagatggacggcaccgaggagctgctggtgaagctgaaccgggaggacctgctgcggaagcagcggaccttcgacaacggcagcatcccccaccagatccacctgggcgagctgcacgccatcctgcggcggcaggaggacttctaccccttcctgaaggacaaccgggagaagatcgagaagatcctgaccttccggatcccctactacgtgggccccctggcccggggcaacagccggttcgcctggatgacccggaagagcgaggagaccatcaccccctggaacttcgaggaggtggtggacaagggcgccagcgcccagagcttcatcgagcggatgaccaacttcgacaagaacctgcccaacgagaaggtgctgcccaagcacagcctgctgtacgagtacttcaccgtgtacaacgagctgaccgccgtgaagtacgtgaccgagggcatgcggaagcccgccttcctgagcggcgagcagaagaaggccatcgtggacctgctgttcaagaccaaccggaaggtgaccgtgaagcagctgaaggaggactacttcaagaagatcgagtgcttcgacagcgtggagatcagcggcgtggaggaccggttcaacgccagcctgggcacctaccacgacctgctgaagatcatcaaggacaaggacttcctggacaacgaggagaacgaggacatcctggaggacatcgtgctgaccctgaccctgttcgaggaccgggagatgatcgaggagcggctgaagacctacgcccacctgttcgacgacaaggtgatgaagcagctgaagcggcggcggtacaccggctggggccggctgagccggaagctgatcaacggcatccgggacaagcagagcggcaagaccatcctggacttcctgaagagcgacggcttcgccaacgccaacttcatggccctgatcgccgacgacagcctgaccttcaaggaggacatccagaaggcccaggtgagcggccagggcgacagcctgcacgagcacatcgccaacctggccggcagccccgccatcaagaagggcatcctgcagaccgtgaaggtggtggacgagctggtgaaggtgatgggccggcacaagcccgagaacatcgtgatcgagatggcccgggagaaccagaccacccagaagggccagaagaacagccgggagcggatgaagcggatcgaggagggcatcaaggagctgggcagccagatcctgaaggagcaccccgtggagaacacccagctgcagaacgagaagctgtacctgtactacctgcagaacggccgggacatgtacgtggaccaggagctggacatcaaccggctgagcgactacgacgtggacgccatcgtgccccagagcttcctgaaggacgacagcatcgacaacaaggtgctgacccggagcgacaagaaccggggcaagagcgacaacgtgcccagcgaggaggtggtgaagaagatgaagaactactggcggcagctgctgaacgccaagctgatcacccagcggaagttcgacaacctgaccaaggccgagcggggcggcctgagcgagctggacaaggccggcttcatcaagcggcagctggtggagacccggcagatcaccaagcacgtggcccagatcctggacagccggatgaacaccaagtacgacgagaacgacaagctgatccgggaggtgaaggtgatcaccctgaagagcaagctggtgagcgacttccggaaggacttccagttctacaaggtgcgggagatcaacaactaccaccacgcccacgacgcctacctgaacgccgtggtgggcaccgccctgatcaagaagtaccccaagctggagagcgagttcgtgtacggcgactacaaggtgtacgacgtgcggaagatgatcgccaagagcgagcaggagatcggcaaggccaccgccaagtacttcttctacagcaacatcatgaacttcttcaagaccgagatcaccctggccaacggcgagatccggaagcggcccctgatcgagaccaacggcgagaccggcgagatcgtgtgggacaagggccgggacttcgccaccgtgcggaaggtgctgagcatgccccaggtgaacatcgtgaagaagaccgaggtgcagaccggcggcttcagcaaggagagcatcctgcccaagcggaacagcgacaagctgatcgcccggaagaaggactgggaccccaagaagtacggcggcttcgacagccccaccgtggcctacagcgtgctggtggtggccaaggtggagaagggcaagagcaagaagctgaagagcgtgaaggagctgctgggcatcaccatcatggagcggagcagcttcgagaagaaccccatcgacttcctggaggccaagggctacaaggaggtgaagaaggacctgatcatcaagctgcccaagtacagcctgttcgagctggagaacggccggaagcggatgctggccagcgccggcgagctgcagaagggcaacgagctggccctgcccagcaagtacgtgaacttcctgtacctggccagccactacgagaagctgaagggcagccccgaggacaacgagcagaagcagctgttcgtggagcagcacaagcactacctggacgagatcatcgagcagatcagcgagttcagcaagcgggtgatcctggccgacgccaacctggacaaggtgctgagcgcctacaacaagcaccgggacaagcccatccgggagcaggccgagaacatcatccacctgttcaccctgaccaacctgggcgcccccgccgccttcaagtacttcgacaccaccatcgaccggaagcggtacaccagcaccaaggaggtgctggacgccaccctgatccaccagagcatcaccggcctgtacgagacccggatcgacctgagccagctgggcggcgaccccaagaagaagcggaaggtggaggaccccaagaagaagcggaaggtgggcggcggcggcggcatggacgccaagagcctgaccgcctggagccggaccctggtgaccttcaaggacgtgttcgtggacttcacccgggaggagtggaagctgctggacaccgcccagcagatcgtgtaccggaacgtgatgctggagaactacaagaacctggtgagcctgggctaccagctgaccaagcccgacgtgatcctgcggctggagaagggcgaggagccctgataataggctggagcctcggtggccatgcttcttgccccttgggcctccccccagcccctcctccccttcctgcacccgtacccccgtggtctttgaataaagtctgagtgggcggcaaaaaaaaaaaaaaaaaaaaaaaaaaaaaaagcatatgactaaaaaaaaaaaaaaaaaaaaaaaaaaaaaaaaaaaaaaaaaaaaaaaaaaaaaaaaaaaaaaaaaaaaaa

SEQ ID NO: 9 - DNA, 10 bp, synthetic construct
  source 1..10: mol_type = other DNA
gccaccatgg

SEQ ID NO: 10 - DNA, 125 bp, synthetic construct
  source 1..125: mol_type = other DNA
gggagacccaagctggctagcgtttaaacttaagcttggtaccgagctcggatccactagtccagtgtggtggaattcgggaaataagagagaaaagaagagtaagaagaaatataagagccacc

SEQ ID NO: 11 - DNA, 47 bp, synthetic construct
  source 1..47: mol_type = other DNA
gggaaataagagagaaaagaagagtaagaagaaatataagagccacc

SEQ ID NO: 12 - DNA, 110 bp, synthetic construct
  source 1..110: mol_type = other DNA
aaaaaaaaaaaaaaaaaaaaaaaaaaaaaagcatatgactaaaaaaaaaaaaaaaaaaaaaaaaaaaaaaaaaaaaaaaaaaaaaaaaaaaaaaaaaaaaaaaaaaaaaa

SEQ ID NO: 13 - DNA, 119 bp, synthetic construct
  source 1..119: mol_type = other DNA
tgataataggctggagcctcggtggccatgcttcttgccccttgggcctccccccagcccctcctccccttcctgcacccgtacccccgtggtctttgaataaagtctgagtgggcggc

SEQ ID NO: 14 - DNA, 100 bp, synthetic construct
  source 1..100: mol_type = other DNA
aaaggctgctgatgacacctgttttagagctagaaatagcaagttaaaataaggctagtccgttatcaacttgaaaaagtggcaccgagtcggtgctttt

SEQ ID NO: 15 - DNA, 100 bp, synthetic construct
  source 1..100: mol_type = other DNA
ataccagtccagcaaggcaggttttagagctagaaatagcaagttaaaataaggctagtccgttatcaacttgaaaaagtggcaccgagtcggtgctttt

SEQ ID NO: 16 - DNA, 100 bp, synthetic construct
  source 1..100: mol_type = other DNA
agtgagtctggagagctgcagttttagagctagaaatagcaagttaaaataaggctagtccgttatcaacttgaaaaagtggcaccgagtcggtgctttt

SEQ ID NO: 17 - DNA, 100 bp, synthetic construct
  source 1..100: mol_type = other DNA
tcacagaaacactcaccgtagttttagagctagaaatagcaagttaaaataaggctagtccgttatcaacttgaaaaagtggcaccgagtcggtgctttt

SEQ ID NO: 18 - DNA, 100 bp, synthetic construct
  source 1..100: mol_type = other DNA
tttgaccatcagaggacactgttttagagctagaaatagcaagttaaaataaggctagtccgttatcaacttgaaaaagtggcaccgagtcggtgctttt

SEQ ID NO: 19 - DNA, 100 bp, synthetic construct
  source 1..100: mol_type = other DNA
aaaggctgctgatgacacctgttttagagctagaaatagcaagttaaaataaggctagtccgttatgaacttgaaaaagtggcaccgagtcggtgctttt

SEQ ID NO: 20 - DNA, 100 bp, synthetic construct
  source 1..100: mol_type = other DNA
aaaggctgctgatgacacctgttttagagctagaaatagcaagttaaaataaggctagtccgtttacaacttgaaaaagtggcaccgagtcggtgctttt

SEQ ID NO: 21 - DNA, 82 bp, synthetic construct
  source 1..82: mol_type = other DNA
aaaggctgctgatgacacctgttttagagctagaaatagcaagttaaaataaggctagtccgttatcaacttgaaaaagtgg

SEQ ID NO: 22 - DNA, 36 bp, synthetic construct
  source 1..36: mol_type = other DNA
aaaggctgctgatgacacctgttttagagctatgct

SEQ ID NO: 23 - DNA, 68 bp, synthetic construct
  source 1..68: mol_type = other DNA
agcatagcaagttaaaataaggctagtccgttatcaacttgaaaaagtggcaccgagtcggtgctttt

SEQ ID NO: 24 - DNA, 20 bp, synthetic construct
  source 1..20: mol_type = other DNA
aaaggctgctgatgacacct

SEQ ID NO: 25 - DNA, 20 bp, synthetic construct
  source 1..20: mol_type = other DNA
ataccagtccagcaaggcag

SEQ ID NO: 26 - DNA, 20 bp, synthetic construct
  source 1..20: mol_type = other DNA
agtgagtctggagagctgca

SEQ ID NO: 27 - DNA, 20 bp, synthetic construct
  source 1..20: mol_type = other DNA
tcacagaaacactcaccgta

SEQ ID NO: 28 - DNA, 20 bp, synthetic construct
  source 1..20: mol_type = other DNA
tttgaccatcagaggacact

SEQ ID NO: 29 - DNA, 20 bp, synthetic construct
  source 1..20: mol_type = other DNA
agagtctctcagctggtaca

SEQ ID NO: 30 - DNA, 20 bp, synthetic construct
  source 1..20: mol_type = other DNA
tcagggttctggatatctgt

SEQ ID NO: 31 - DNA, 20 bp, synthetic construct
  source 1..20: mol_type = other DNA
ctggatatctgtgggacaag

SEQ ID NO: 32 - DNA, 20 bp, synthetic construct
  source 1..20: mol_type = other DNA
acgacgcgtgggtggcaagc

SEQ ID NO: 33 - DNA, 20 bp, synthetic construct
  source 1..20: mol_type = other DNA
gagtccgagcagaagaagaa

SEQ ID NO: 34 - DNA, 20 bp, synthetic construct
  source 1..20: mol_type = other DNA
ggtgagtgagtgtgtgcgtg

SEQ ID NO: 35 - DNA, 20 bp, synthetic construct
  source 1..20: mol_type = other DNA
gaacacaaagcatagactgc

SEQ ID NO: 36 - DNA, 20 bp, synthetic construct
  source 1..20: mol_type = other DNA
gccatcctgccaagaatgag

SEQ ID NO: 37 - DNA, 20 bp, synthetic construct
  source 1..20: mol_type = other DNA
cccgcaccttggcgcagcgg

SEQ ID NO: 38 - DNA, 20 bp, synthetic construct
  source 1..20: mol_type = other DNA
gagtatgaggcatagactgc

SEQ ID NO: 39 - DNA, 20 bp, synthetic construct
  source 1..20: mol_type = other DNA
tataggaaaaccagtgagtc

SEQ ID NO: 40 - DNA, 20 bp, synthetic construct
  source 1..20: mol_type = other DNA
gggaaagacccagcatccgt

SEQ ID NO: 41 - DNA, 20 bp, synthetic construct
  source 1..20: mol_type = other DNA
gaacacaaagcatagactgc

SEQ ID NO: 42 - DNA, 20 bp, synthetic construct
  source 1..20: mol_type = other DNA
ggcccagactgagcacgtga

SEQ ID NO: 43 - DNA, 20 bp, synthetic construct
  source 1..20: mol_type = other DNA
ggcactgcggctggaggtgg

SEQ ID NO: 44 - DNA, 20 bp, synthetic construct
  source 1..20: mol_type = other DNA
gcggaaaccttctagggtgt

SEQ ID NO: 45 - DNA, 20 bp, synthetic construct
  source 1..20: mol_type = other DNA
aggagttccgcagtatggat

SEQ ID NO: 46 - DNA, 20 bp, synthetic construct
  source 1..20: mol_type = other DNA
cagatgagaaggcacagacg

SEQ ID NO: 47 - DNA, 20 bp, synthetic construct
  source 1..20: mol_type = other DNA
gagtctaagcagaagaagaa

SEQ ID NO: 48 - DNA, 20 bp, synthetic construct
  source 1..20: mol_type = other DNA
gaggccgagcagaagaaaga

SEQ ID NO: 49 - DNA, 21 bp, synthetic construct
  source 1..21: mol_type = other DNA
gtgtgagtaagtgtgtgtgtg

SEQ ID NO: 50 - DNA, 20 bp, synthetic construct
  source 1..20: mol_type = other DNA
ggtgagtgtgtgtgtgcatg

SEQ ID NO: 51 - DNA, 20 bp, synthetic construct
  source 1..20: mol_type = other DNA
tagaggaaaaccagtcagtc

SEQ ID NO: 52 - DNA, 20 bp, synthetic construct
  source 1..20: mol_type = other DNA
cataggaaaaccagtgagtt

SEQ ID NO: 53 - DNA, 20 bp, synthetic construct
  source 1..20: mol_type = other DNA
taaaggaaaaccagtgggtc

SEQ ID NO: 54 - DNA, 20 bp, synthetic construct
  source 1..20: mol_type = other DNA
gggaaagtcccagcatcctt

SEQ ID NO: 55 - DNA, 20 bp, synthetic construct
  source 1..20: mol_type = other DNA
gggaaaagcccagcatccct

SEQ ID NO: 56 - DNA, 20 bp, synthetic construct
  source 1..20: mol_type = other DNA
gggaaggacccagcatcctg

SEQ ID NO: 57 - DNA, 20 bp, synthetic construct
  source 1..20: mol_type = other DNA
gaacacaatgcatagattgc

SEQ ID NO: 58 - DNA, 20 bp, synthetic construct
  source 1..20: mol_type = other DNA
gaaacaaaagcatagactgc

SEQ ID NO: 59 - DNA, 20 bp, synthetic construct
  source 1..20: mol_type = other DNA
gaacacaaggcagagactgt

SEQ ID NO: 60 - DNA, 20 bp, synthetic construct
  source 1..20: mol_type = other DNA
cacccagactgagcacgtgc

SEQ ID NO: 61 - DNA, 20 bp, synthetic construct
  source 1..20: mol_type = other DNA
gacacagactgggcacgtga

SEQ ID NO: 62 - DNA, 20 bp, synthetic construct
  source 1..20: mol_type = other DNA
tgcactgcggccggaggagg

SEQ ID NO: 63 - DNA, 20 bp, synthetic construct
  source 1..20: mol_type = other DNA
ggcatcacggctggaggtgg

SEQ ID NO: 64 - DNA, 20 bp, synthetic construct
  source 1..20: mol_type = other DNA
ggcgctgcggcgggaggtgg

SEQ ID NO: 65 - protein, 1400 aa, synthetic construct
MAPKKKRKVGIHGVPAADKKYSIGLDIGTNSVGWAVITDEYKVPSKKFKVLGNTDRHSIKKNLIGALLFDSGETAEATRLKRTARRRYTRRKNRICYLQEIFSNEMAKVDDSFFHRLEESFLVEEDKKHERHPIFGNIVDEVAYHEKYPTIYHLRKKLVDSTDKADLRLIYLALAHMIKFRGHFLIEGDLNPDNSDVDKLFIQLVQTYNQLFEENPINASGVDAKAILSARLSKSRRLENLIAQLPGEKKNGLFGNLIALSLGLTPNFKSNFDLAEDAKLQLSKDTYDDDLDNLLAQIGDQYADLFLAAKNLSDAILLSDILRVNTEITKAPLSASMIKRYDEHHQDLTLLKALVRQQLPEKYKEIFFDQSKNGYAGYIDGGASQEEFYKFIKPILEKMDGTEELLVKLNREDLLRKQRTFDNGSIPHQIHLGELHAILRRQEDFYPFLKDNREKIEKILTFRIPYYVGPLARGNSRFAWMTRKSEETITPWNFEEVVDKGASAQSFIERMTNFDKNLPNEKVLPKHSLLYEYFTVYNELTKVKYVTEGMRKPAFLSGEQKKAIVDLLFKTNRKVTVKQLKEDYFKKIECFDSVEISGVEDRFNASLGTYHDLLKIIKDKDFLDNEENEDILEDIVLTLTLFEDREMIEERLKTYAHLFDDKVMKQLKRRRYTGWGRLSRKLINGIRDKQSGKTILDFLKSDGFANRNFMQLIHDDSLTFKEDIQKAQVSGQGDSLHEHIANLAGSPAIKKGILQTVKVVDELVKVMGRHKPENIVIEMARENQTTQKGQKNSRERMKRIEEGIKELGSQILKEHPVENTQLQNEKLYLYYLQNGRDMYVDQELDINRLSDYDVDHIVPQSFLKDDSIDNKVLTRSDKNRGKSDNVPSEEVVKKMKNYWRQLLNAKLITQRKFDNLTKAERGGLSELDKAGFIKRQLVETRQITKHVAQILDSRMNTKYDENDKLIREVKVITLKSKLVSDFRKDFQFYKVREINNYHHAHDAYLNAVVGTALIKKYPKLESEFVYGDYKVYDVRKMIAKSEQEIGKATAKYFFYSNIMNFFKTEITLANGEIRKRPLIETNGETGEIVWDKGRDFATVRKVLSMPQVNIVKKTEVQTGGFSKESILPKRNSDKLIARKKDWDPKKYGGFDSPTVAYSVLVVAKVEKGKSKKLKSVKELLGITIMERSSFEKNPIDFLEAKGYKEVKKDLIIKLPKYSLFELENGRKRMLASAGELQKGNELALPSKYVNFLYLASHYEKLKGSPEDNEQKQLFVEQHKHYLDEIIEQISEFSKRVILADANLDKVLSAYNKHRDKPIREQAENIIHLFTLTNLGAPAAFKYFDTTIDRKRYTSTKEVLDATLIHQSITGLYETRIDLSQLGGDKRPAATKKAGQAKKKK

SEQ ID NO: 66 - protein, 1400 aa, synthetic construct
MAPKKKRKVGIHGVPAADKKYSIGLDIGTNSVGWAVITDEYKVPSKKFKVLGNTDRHSIKKNLIGALLFDSGETAEATRLKRTARRRYTRRKNRICYLQEIFSNEMAKVDDSFFHRLEESFLVEEDKKHERHPIFGNIVDEVAYHEKYPTIYHLRKKLVDSTDKADLRLIYLALAHMIKFRGHFLIEGDLNPDNSDVDKLFIQLVQTYNQLFEENPINASGVDAKAILSARLSKSRRLENLIAQLPGEKKNGLFGNLIALSLGLTPNFKSNFDLAEDAKLQLSKDTYDDDLDNLLAQIGDQYADLFLAAKNLSDAILLSDILRVNTEITKAPLSASMIKRYDEHHQDLTLLKALVRQQLPEKYKEIFFDQSKNGYAGYIDGGASQEEFYKFIKPILEKMDGTEELLVKLNREDLLRKQRTFDNGSIPHQIHLGELHAILRRQEDFYPFLKDNREKIEKILTFRIPYYVGPLARGNSRFAWMTRKSEETITPWNFEEVVDKGASAQSFIERMTNFDKNLPNEKVLPKHSLLYEYFTVYNELTAVKYVTEGMRKPAFLSGEQKKAIVDLLFKTNRKVTVKQLKEDYFKKIECFDSVEISGVEDRFNASLGTYHDLLKIIKDKDFLDNEENEDILEDIVLTLTLFEDREMIEERLKTYAHLFDDKVMKQLKRRRYTGWGRLSRKLINGIRDKQSGKTILDFLKSDGFANANFMALIADDSLTFKEDIQKAQVSGQGDSLHEHIANLAGSPAIKKGILQTVKVVDELVKVMGRHKPENIVIEMARENQTTQKGQKNSRERMKRIEEGIKELGSQILKEHPVENTQLQNEKLYLYYLQNGRDMYVDQELDINRLSDYDVDHIVPQSFLKDDSIDNKVLTRSDKNRGKSDNVPSEEVVKKMKNYWRQLLNAKLITQRKFDNLTKAERGGLSELDKAGFIKRQLVETRQITKHVAQILDSRMNTKYDENDKLIREVKVITLKSKLVSDFRKDFQFYKVREINNYHHAHDAYLNAVVGTALIKKYPKLESEFVYGDYKVYDVRKMIAKSEQEIGKATAKYFFYSNIMNFFKTEITLANGEIRKRPLIETNGETGEIVWDKGRDFATVRKVLSMPQVNIVKKTEVQTGGFSKESILPKRNSDKLIARKKDWDPKKYGGFDSPTVAYSVLVVAKVEKGKSKKLKSVKELLGITIMERSSFEKNPIDFLEAKGYKEVKKDLIIKLPKYSLFELENGRKRMLASAGELQKGNELALPSKYVNFLYLASHYEKLKGSPEDNEQKQLFVEQHKHYLDEIIEQISEFSKRVILADANLDKVLSAYNKHRDKPIREQAENIIHLFTLTNLGAPAAFKYFDTTIDRKRYTSTKEVLDATLIHQSITGLYETRIDLSQLGGDKRPAATKKAGQAKKKK

SEQ ID NO: 67 - protein, 1400 aa, synthetic construct
MAPKKKRKVGIHGVPAADKKYSIGLDIGTNSVGWAVITDEYKVPSKKFKVLGNTDRHSIKKNLIGALLFDSGETAEATRLKRTARRRYTRRKNRICYLQEIFSNEMAKVDDSFFHRLEESFLVEEDKKHERHPIFGNIVDEVAYHEKYPTIYHLRKKLVDSTDKADLRLIYLALAHMIKFRGHFLIEGDLNPDNSDVDKLFIQLVQTYNQLFEENPINASGVDAKAILSARLSKSRRLENLIAQLPGEKKNGLFGNLIALSLGLTPNFKSNFDLAEDAKLQLSKDTYDDDLDNLLAQIGDQYADLFLAAKNLSDAILLSDILRVNTEITKAPLSASMIKRYDEHHQDLTLLKALVRQQLPEKYKEIFFDQSKNGYAGYIDGGASQEEFYKFIKPILEKMDGTEELLVKLNREDLLRKQRTFDNGSIPHQIHLGELHAILRRQEDFYPFLKDNREKIEKILTFRIPYYVGPLARGNSRFAWMTRKSEETITPWNFEEVVDKGASAQSFIERMTAFDKNLPNEKVLPKHSLLYEYFTVYNELTKVKYVTEGMRKPAFLSGEQKKAIVDLLFKTNRKVTVKQLKEDYFKKIECFDSVEISGVEDRFNASLGTYHDLLKIIKDKDFLDNEENEDILEDIVLTLTLFEDREMIEERLKTYAHLFDDKVMKQLKRRRYTGWGALSRKLINGIRDKQSGKTILDFLKSDGFANRNFMALIHDDSLTFKEDIQKAQVSGQGDSLHEHIANLAGSPAIKKGILQTVKVVDELVKVMGRHKPENIVIEMARENQTTQKGQKNSRERMKRIEEGIKELGSQILKEHPVENTQLQNEKLYLYYLQNGRDMYVDQELDINRLSDYDVDHIVPQSFLKDDSIDNKVLTRSDKNRGKSDNVPSEEVVKKMKNYWRQLLNAKLITQRKFDNLTKAERGGLSELDKAGFIKRQLVETRAITKHVAQILDSRMNTKYDENDKLIREVKVITLKSKLVSDFRKDFQFYKVREINNYHHAHDAYLNAVVGTALIKKYPKLESEFVYGDYKVYDVRKMIAKSEQEIGKATAKYFFYSNIMNFFKTEITLANGEIRKRPLIETNGETGEIVWDKGRDFATVRKVLSMPQVNIVKKTEVQTGGFSKESILPKRNSDKLIARKKDWDPKKYGGFDSPTVAYSVLVVAKVEKGKSKKLKSVKELLGITIMERSSFEKNPIDFLEAKGYKEVKKDLIIKLPKYSLFELENGRKRMLASAGELQKGNELALPSKYVNFLYLASHYEKLKGSPEDNEQKQLFVEQHKHYLDEIIEQISEFSKRVILADANLDKVLSAYNKHRDKPIREQAENIIHLFTLTNLGAPAAFKYFDTTIDRKRYTSTKEVLDATLIHQSITGLYETRIDLSQLGGDKRPAATKKAGQAKKKK

SEQ ID NO: 68 - protein, 1368 aa, synthetic construct [sequence omitted]

SEQ ID NO: 69 - protein, 1368 aa, synthetic construct
ADKKYSIGLDIGTNSVGWAVITDEYKVPSKKFKVLGNTDRHSIKKNLIGALLFDSGETAEATRLKRTARRRYTRRKNRICYLQEIFSNEMAKVDDSFFHRLEESFLVEEDKKHERHPIFGNIVDEVAYHEKYPTIYHLRKKLVDSTDKADLRLIYLALAHMIKFRGHFLIEGDLNPDNSDVDKLFIQLVQTYNQLFEENPINASGVDAKAILSARLSKSRRLENLIAQLPGEKKNGLFGNLIALSLGLTPNFKSNFDLAEDAKLQLSKDTYDDDLDNLLAQIGDQYADLFLAAKNLSDAILLSDILRVNTEITKAPLSASMIKRYDEHHQDLTLLKALVRQQLPEKYKEIFFDQSKNGYAGYIDGGASQEEFYKFIKPILEKMDGTEELLVKLNREDLLRKQRTFDNGSIPHQIHLGELHAILRRQEDFYPFLKDNREKIEKILTFRIPYYVGPLARGNSRFAWMTRKSEETITPWNFEEVVDKGASAQSFIERMTNFDKNLPNEKVLPKHSLLYEYFTVYNELTAVKYVTEGMRKPAFLSGEQKKAIVDLLFKTNRKVTVKQLKEDYFKKIECFDSVEISGVEDRFNASLGTYHDLLKIIKDKDFLDNEENEDILEDIVLTLTLFEDREMIEERLKTYAHLFDDKVMKQLKRRRYTGWGRLSRKLINGIRDKQSGKTILDFLKSDGFANANFMALIADDSLTFKEDIQKAQVSGQGDSLHEHIANLAGSPAIKKGILQTVKVVDELVKVMGRHKPENIVIEMARENQTTQKGQKNSRERMKRIEEGIKELGSQILKEHPVENTQLQNEKLYLYYLQNGRDMYVDQELDINRLSDYDVDHIVPQSFLKDDSIDNKVLTRSDKNRGKSDNVPSEEVVKKMKNYWRQLLNAKLITQRKFDNLTKAERGGLSELDKAGFIKRQLVETRQITKHVAQILDSRMNTKYDENDKLIREVKVITLKSKLVSDFRKDFQFYKVREINNYHHAHDAYLNAVVGTALIKKYPKLESEFVYGDYKVYDVRKMIAKSEQEIGKATAKYFFYSNIMNFFKTEITLANGEIRKRPLIETNGETGEIVWDKGRDFATVRKVLSMPQVNIVKKTEVQTGGFSKESILPKRNSDKLIARKKDWDPKKYGGFDSPTVAYSVLVVAKVEKGKSKKLKSVKELLGITIMERSSFEKNPIDFLEAKGYKEVKKDLIIKLPKYSLFELENGRKRMLASAGELQKGNELALPSKYVNFLYLASHYEKLKGSPEDNEQKQLFVEQHKHYLDEIIEQISEFSKRVILADANLDKVLSAYNKHRDKPIREQAENIIHLFTLTNLGAPAAFKYFDTTIDRKRYTSTKEVLDATLIHQSITGLYETRIDLSQLGGD

SEQ ID NO: 70 - protein, 16 aa, synthetic construct
KRPAATKKAGQAKKKK

SEQ ID NO: 71 - protein, 16 aa, synthetic construct
APKKKRKVGIHGVPAA

SEQ ID NO: 72 - protein, 1605 aa, synthetic construct
MKRTADGSEFESPKKKRKVSEVEFSHEYWMRHALTLAKRARDEREVPVGAVLVLNNRVIGEGWNRAIGLHDPTAHAEIMALRQGGLVMQNYRLIDATLYVTFEPCVMCAGAMIHSRIGRVVFGVRNSKRGAAGSLMNVLNYPGMNHRVEITEGILADECAALLCDFYRMPRQVFNAQKKAQSSINSGGSSGGSSGSETPGTSESATPESSGGSSGGSDKKYSIGLAIGTNSVGWAVITDEYKVPSKKFKVLGNTDRHSIKKNLIGALLFDSGETAEATRLKRTARRRYTRRKNRICYLQEIFSNEMAKVDDSFFHRLEESFLVEEDKKHERHPIFGNIVDEVAYHEKYPTIYHLRKKLVDSTDKADLRLIYLALAHMIKFRGHFLIEGDLNPDNSDVDKLFIQLVQTYNQLFEENPINASGVDAKAILSARLSKSRRLENLIAQLPGEKKNGLFGNLIALSLGLTPNFKSNFDLAEDAKLQLSKDTYDDDLDNLLAQIGDQYADLFLAAKNLSDAILLSDILRVNTEITKAPLSASMIKRYDEHHQDLTLLKALVRQQLPEKYKEIFFDQSKNGYAGYIDGGASQEEFYKFIKPILEKMDGTEELLVKLNREDLLRKQRTFDNGSIPHQIHLGELHAILRRQEDFYPFLKDNREKIEKILTFRIPYYVGPLARGNSRFAWMTRKSEETITPWNFEEVVDKGASAQSFIERMTNFDKNLPNEKVLPKHSLLYEYFTVYNELTKVKYVTEGMRKPAFLSGEQKKAIVDLLFKTNRKVTVKQLKEDYFKKIECFDSVEISGVEDRFNASLGTYHDLLKIIKDKDFLDNEENEDILEDIVLTLTLFEDREMIEERLKTYAHLFDDKVMKQLKRRRYTGWGRLSRKLINGIRDKQSGKTILDFLKSDGFANRNFMQLIHDDSLTFKEDIQKAQVSGQGDSLHEHIANLAGSPAIKKGILQTVKVVDELVKVMGRHKPENIVIEMARENQTTQKGQKNSRERMKRIEEGIKELGSQILKEHPVENTQLQNEKLYLYYLQNGRDMYVDQELDINRLSDYDVDHIVPQSFLKDDSIDNKVLTRSDKNRGKSDNVPSEEVVKKMKNYWRQLLNAKLITQRKFDNLTKAERGGLSELDKAGFIKRQLVETRQITKHVAQILDSRMNTKYDENDKLIREVKVITLKSKLVSDFRKDFQFYKVREINNYHHAHDAYLNAVVGTALIKKYPKLESEFVYGDYKVYDVRKMIAKSEQEIGKATAKYFFYSNIMNFFKTEITLANGEIRKRPLIETNGETGEIVWDKGRDFATVRKVLSMPQVNIVKKTEVQTGGFSKESILPKRNSDKLIARKKDWDPKKYGGFDSPTVAYSVLVVAKVEKGKSKKLKSVKELLGITIMERSSFEKNPIDFLEAKGYKEVKKDLIIKLPKYSLFELENGRKRMLASAGELQKGNELALPSKYVNFLYLASHYEKLKGSPEDNEQKQLFVEQHKHYLDEIIEQISEFSKRVILADANLDKVLSAYNKHRDKPIREQAENIIHLFTLTNLGAPAAFKYFDTTIDRKRYTSTKEVLDATLIHQSITGLYETRIDLSQLGGDSGGSKRTADGSEFEPKKKRKV

SEQ ID NO: 73 - protein, 1605 aa, synthetic construct
MKRTADGSEFESPKKKRKVSEVEFSHEYWMRHALTLAKRARDEREVPVGAVLVLNNRVIGEGWNRAIGLHDPTAHAEIMALRQGGLVMQNYRLIDATLYVTFEPCVMCAGAMIHSRIGRVVFGVRNSKRGAAGSLMNVLNYPGMNHRVEITEGILADECAALLCDFYRMPRQVFNAQKKAQSSINSGGSSGGSSGSETPGTSESATPESSGGSSGGSDKKYSIGLAIGTNSVGWAVITDEYKVPSKKFKVLGNTDRHSIKKNLIGALLFDSGETAEATRLKRTARRRYTRRKNRICYLQEIFSNEMAKVDDSFFHRLEESFLVEEDKKHERHPIFGNIVDEVAYHEKYPTIYHLRKKLVDSTDKADLRLIYLALAHMIKFRGHFLIEGDLNPDNSDVDKLFIQLVQTYNQLFEENPINASGVDAKAILSARLSKSRRLENLIAQLPGEKKNGLFGNLIALSLGLTPNFKSNFDLAEDAKLQLSKDTYDDDLDNLLAQIGDQYADLFLAAKNLSDAILLSDILRVNTEITKAPLSASMIKRYDEHHQDLTLLKALVRQQLPEKYKEIFFDQSKNGYAGYIDGGASQEEFYKFIKPILEKMDGTEELLVKLNREDLLRKQRTFDNGSIPHQIHLGELHAILRRQEDFYPFLKDNREKIEKILTFRIPYYVGPLARGNSRFAWMTRKSEETITPWNFEEVVDKGASAQSFIERMTNFDKNLPNEKVLPKHSLLYEYFTVYNELTAVKYVTEGMRKPAFLSGEQKKAIVDLLFKTNRKVTVKQLKEDYFKKIECFDSVEISGVEDRFNASLGTYHDLLKIIKDKDFLDNEENEDILEDIVLTLTLFEDREMIEERLKTYAHLFDDKVMKQLKRRRYTGWGRLSRKLINGIRDKQSGKTILDFLKSDGFANANFMALIADDSLTFKEDIQKAQVSGQGDSLHEHIANLAGSPAIKKGILQTVKVVDELVKVMGRHKPENIVIEMARENQTTQKGQKNSRERMKRIEEGIKELGSQILKEHPVENTQLQNEKLYLYYLQNGRDMYVDQELDINRLSDYDVDHIVPQSFLKDDSIDNKVLTRSDKNRGKSDNVPSEEVVKKMKNYWRQLLNAKLITQRKFDNLTKAERGGLSELDKAGFIKRQLVETRQITKHVAQILDSRMNTKYDENDKLIREVKVITLKSKLVSDFRKDFQFYKVREINNYHHAHDAYLNAVVGTALIKKYPKLESEFVYGDYKVYDVRKMIAKSEQEIGKATAKYFFYSNIMNFFKTEITLANGEIRKRPLIETNGETGEIVWDKGRDFATVRKVLSMPQVNIVKKTEVQTGGFSKESILPKRNSDKLIARKKDWDPKKYGGFDSPTVAYSVLVVAKVEKGKSKKLKSVKELLGITIMERSSFEKNPIDFLEAKGYKEVKKDLIIKLPKYSLFELENGRKRMLASAGELQKGNELALPSKYVNFLYLASHYEKLKGSPEDNEQKQLFVEQHKHYLDEIIEQISEFSKRVILADANLDKVLSAYNKHRDKPIREQAENIIHLFTLTNLGAPAAFKYFDTTIDRKRYTSTKEVLDATLIHQSITGLYETRIDLSQLGGDSGGSKRTADGSEFEPKKKRKV

SEQ ID NO: 74 - protein, 18 aa, synthetic construct
KRTADGSEFESPKKKRKV

SEQ ID NO: 75 - protein, 17 aa, synthetic construct
KRTADGSEFEPKKKRKV

SEQ ID NO: 76 - protein, 166 aa, synthetic construct
SEVEFSHEYWMRHALTLAKRARDEREVPVGAVLVLNNRVIGEGWNRAIGLHDPTAHAEIMALRQGGLVMQNYRLIDATLYVTFEPCVMCAGAMIHSRIGRVVFGVRNSKRGAAGSLMNVLNYPGMNHRVEITEGILADECAALLCDFYRMPRQVFNAQKKAQSSIN

SEQ ID NO: 77 - protein, 32 aa, synthetic construct
SGGSSGGSSGSETPGTSESATPESSGGSSGGS

SEQ ID NO: 78 - protein, 1367 aa, synthetic construct
DKKYSIGLAIGTNSVGWAVITDEYKVPSKKFKVLGNTDRHSIKKNLIGALLFDSGETAEATRLKRTARRRYTRRKNRICYLQEIFSNEMAKVDDSFFHRLEESFLVEEDKKHERHPIFGNIVDEVAYHEKYPTIYHLRKKLVDSTDKADLRLIYLALAHMIKFRGHFLIEGDLNPDNSDVDKLFIQLVQTYNQLFEENPINASGVDAKAILSARLSKSRRLENLIAQLPGEKKNGLFGNLIALSLGLTPNFKSNFDLAEDAKLQLSKDTYDDDLDNLLAQIGDQYADLFLAAKNLSDAILLSDILRVNTEITKAPLSASMIKRYDEHHQDLTLLKALVRQQLPEKYKEIFFDQSKNGYAGYIDGGASQEEFYKFIKPILEKMDGTEELLVKLNREDLLRKQRTFDNGSIPHQIHLGELHAILRRQEDFYPFLKDNREKIEKILTFRIPYYVGPLARGNSRFAWMTRKSEETITPWNFEEVVDKGASAQSFIERMTNFDKNLPNEKVLPKHSLLYEYFTVYNELTAVKYVTEGMRKPAFLSGEQKKAIVDLLFKTNRKVTVKQLKEDYFKKIECFDSVEISGVEDRFNASLGTYHDLLKIIKDKDFLDNEENEDILEDIVLTLTLFEDREMIEERLKTYAHLFDDKVMKQLKRRRYTGWGRLSRKLINGIRDKQSGKTILDFLKSDGFANANFMALIADDSLTFKEDIQKAQVSGQGDSLHEHIANLAGSPAIKKGILQTVKVVDELVKVMGRHKPENIVIEMARENQTTQKGQKNSRERMKRIEEGIKELGSQILKEHPVENTQLQNEKLYLYYLQNGRDMYVDQELDINRLSDYDVDHIVPQSFLKDDSIDNKVLTRSDKNRGKSDNVPSEEVVKKMKNYWRQLLNAKLITQRKFDNLTKAERGGLSELDKAGFIKRQLVETRQITKHVAQILDSRMNTKYDENDKLIREVKVITLKSKLVSDFRKDFQFYKVREINNYHHAHDAYLNAVVGTALIKKYPKLESEFVYGDYKVYDVRKMIAKSEQEIGKATAKYFFYSNIMNFFKTEITLANGEIRKRPLIETNGETGEIVWDKGRDFATVRKVLSMPQVNIVKKTEVQTGGFSKESILPKRNSDKLIARKKDWDPKKYGGFDSPTVAYSVLVVAKVEKGKSKKLKSVKELLGITIMERSSFEKNPIDFLEAKGYKEVKKDLIIKLPKYSLFELENGRKRMLASAGELQKGNELALPSKYVNFLYLASHYEKLKGSPEDNEQKQLFVEQHKHYLDEIIEQISEFSKRVILADANLDKVLSAYNKHRDKPIREQAENIIHLFTLTNLGAPAAFKYFDTTIDRKRYTSTKEVLDATLIHQSITGLYETRIDLSQLGGD

SEQ ID NO: 79 - protein, 2085 aa, synthetic construct
MNHDQEFDPPKVYPPVPAEKRKPIRVLSLFDGIATGLLVLKDLGIQVDRYIASEVCEDSITVGMVRHQGKIMYVGDVRSVTQKHIQEWGPFDLVIGGSPCNDLSIVNPARKGLYEGTGRLFFEFYRLLHDARPKEGDDRPFFWLFENVVAMGVSDKRDISRFLESNPVMIDAKEVSAAHRARYFWGNLPGMNRPLASTVNDKLELQECLEHGRIAKFSKVRTITTRSNSIKQGKDQHFPVFMNEKEDILWCTEMERVFGFPVHYTDVSNMSRLARQRLLGRSWSVPVIRHLFAPLKEYFACVSSGNSNANSRGPSFSSGLVPLSLRGSHMGPMEIYKTVSAWKRQPVRVLSLFRNIDKVLKSLGFLESGSGSGGGTLKYVEDVTNVVRRDVEKWGPFDLVYGSTQPLGSSCDRCPGWYMFQFHRILQYALPRQESQRPFFWIFMDNLLLTEDDQETTTRFLQTEAVTLQDVRGRDYQNAMRVWSNIPGLKSKHAPLTPKEEEYLQAQVRSRSKLDAPKVDLLVKNCLLPLREYFKYFSQNSLPLGGPSSGAPPPSGGSPAGSPTSTEEGTSESATPESGPGTSTEPSEGSAPGSPAGSPTSTEEGTSTEPSEGSAPGTSTEPSEMDKKYSIGLAIGTNSVGWAVITDEYKVPSKKFKVLGNTDRHSIKKNLIGALLFDSGETAEATRLKRTARRRYTRRKNRICYLQEIFSNEMAKVDDSFFHRLEESFLVEEDKKHERHPIFGNIVDEVAYHEKYPTIYHLRKKLVDSTDKADLRLIYLALAHMIKFRGHFLIEGDLNPDNSDVDKLFIQLVQTYNQLFEENPINASGVDAKAILSARLSKSRRLENLIAQLPGEKKNGLFGNLIALSLGLTPNFKSNFDLAEDAKLQLSKDTYDDDLDNLLAQIGDQYADLFLAAKNLSDAILLSDILRVNTEITKAPLSASMIKRYDEHHQDLTLLKALVRQQLPEKYKEIFFDQSKNGYAGYIDGGASQEEFYKFIKPILEKMDGTEELLVKLNREDLLRKQRTFDNGSIPHQIHLGELHAILRRQEDFYPFLKDNREKIEKILTFRIPYYVGPLARGNSRFAWMTRKSEETITPWNFEEVVDKGASAQSFIERMTNFDKNLPNEKVLPKHSLLYEYFTVYNELTKVKYVTEGMRKPAFLSGEQKKAIVDLLFKTNRKVTVKQLKEDYFKKIECFDSVEISGVEDRFNASLGTYHDLLKIIKDKDFLDNEENEDILEDIVLTLTLFEDREMIEERLKTYAHLFDDKVMKQLKRRRYTGWGRLSRKLINGIRDKQSGKTILDFLKSDGFANRNFMQLIHDDSLTFKEDIQKAQVSGQGDSLHEHIANLAGSPAIKKGILQTVKVVDELVKVMGRHKPENIVIEMARENQTTQKGQKNSRERMKRIEEGIKELGSQILKEHPVENTQLQNEKLYLYYLQNGRDMYVDQELDINRLSDYDVDAIVPQSFLKDDSIDNKVLTRSDKNRGKSDNVPSEEVVKKMKNYWRQLLNAKLITQRKFDNLTKAERGGLSELDKAGFIKRQLVETRQITKHVAQILDSRMNTKYDENDKLIREVKVITLKSKLVSDFRKDFQFYKVREINNYHHAHDAYLNAVVGTALIKKYPKLESEFVYGDYKVYDVRKMIAKSEQEIGKATAKYFFYSNIMNFFKTEITLANGEIRKRPLIETNGETGEIVWDKGRDFATVRKVLSMPQVNIVKKTEVQTGGFSKESILPKRNSDKLIARKKDWDPKKYGGFDSPTVAYSVLVVAKVEKGKSKKLKSVKELLGITIMERSSFEKNPIDFLEAKGYKEVKKDLIIKLPKYSLFELENGRKRMLASAGELQKGNELALPSKYVNFLYLASHYEKLKGSPEDNEQKQLFVEQHKHYLDEIIEQISEFSKRVILADANLDKVLSAYNKHRDKPIREQAENIIHLFTLTNLGAPAAFKYFDTTIDRKRYTSTKEVLDATLIHQSITGLYETRIDLSQLGGDPKKKRKVEDPKKKRKVGGGGGMDAKSLTAWSRTLVTFKDVFVDFTREEWKLLDTAQQIVYRNVMLENYKNLVSLGYQLTKPDVILRLEKGEEP

SEQ ID NO: 80 - protein, 2085 aa, synthetic construct
MNHDQEFDPPKVYPPVPAEKRKPIRVLSLFDGIATGLLVLKDLGIQVDRYIASEVCEDSITVGMVRHQGKIMYVGDVRSVTQKHIQEWGPFDLVIGGSPCNDLSIVNPARKGLYEGTGRLFFEFYRLLHDARPKEGDDRPFFWLFENVVAMGVSDKRDISRFLESNPVMIDAKEVSAAHRARYFWGNLPGMNRPLASTVNDKLELQECLEHGRIAKFSKVRTITTRSNSIKQGKDQHFPVFMNEKEDILWCTEMERVFGFPVHYTDVSNMSRLARQRLLGRSWSVPVIRHLFAPLKEYFACVSSGNSNANSRGPSFSSGLVPLSLRGSHMGPMEIYKTVSAWKRQPVRVLSLFRNIDKVLKSLGFLESGSGSGGGTLKYVEDVTNVVRRDVEKWGPFDLVYGSTQPLGSSCDRCPGWYMFQFHRILQYALPRQESQRPFFWIFMDNLLLTEDDQETTTRFLQTEAVTLQDVRGRDYQNAMRVWSNIPGLKSKHAPLTPKEEEYLQAQVRSRSKLDAPKVDLLVKNCLLPLREYFKYFSQNSLPLGGPSSGAPPPSGGSPAGSPTSTEEGTSESATPESGPGTSTEPSEGSAPGSPAGSPTSTEEGTSTEPSEGSAPGTSTEPSEMDKKYSIGLAIGTNSVGWAVITDEYKVPSKKFKVLGNTDRHSIKKNLIGALLFDSGETAEATRLKRTARRRYTRRKNRICYLQEIFSNEMAKVDDSFFHRLEESFLVEEDKKHERHPIFGNIVDEVAYHEKYPTIYHLRKKLVDSTDKADLRLIYLALAHMIKFRGHFLIEGDLNPDNSDVDKLFIQLVQTYNQLFEENPINASGVDAKAILSARLSKSRRLENLIAQLPGEKKNGLFGNLIALSLGLTPNFKSNFDLAEDAKLQLSKDTYDDDLDNLLAQIGDQYADLFLAAKNLSDAILLSDILRVNTEITKAPLSASMIKRYDEHHQDLTLLKALVRQQLPEKYKEIFFDQSKNGYAGYIDGGASQEEFYKFIKPILEKMDGTEELLVKLNREDLLRKQRTFDNGSIPHQIHLGELHAILRRQEDFYPFLKDNREKIEKILTFRIPYYVGPLARGNSRFAWMTRKSEETITPWNFEEVVDKGASAQSFIERMTNFDKNLPNEKVLPKHSLLYEYFTVYNELTAVKYVTEGMRKPAFLSGEQKKAIVDLLFKTNRKVTVKQLKEDYFKKIECFDSVEISGVEDRFNASLGTYHDLLKIIKDKDFLDNEENEDILEDIVLTLTLFEDREMIEERLKTYAHLFDDKVMKQLKRRRYTGWGRLSRKLINGIRDKQSGKTILDFLKSDGFANANFMALIADDSLTFKEDIQKAQVSGQGDSLHEHIANLAGSPAIKKGILQTVKVVDELVKVMGRHKPENIVIEMARENQTTQKGQKNSRERMKRIEEGIKELGSQILKEHPVENTQLQNEKLYLYYLQNGRDMYVDQELDINRLSDYDVDAIVPQSFLKDDSIDNKVLTRSDKNRGKSDNVPSEEVVKKMKNYWRQLLNAKLITQRKFDNLTKAERGGLSELDKAGFIKRQLVETRQITKHVAQILDSRMNTKYDENDKLIREVKVITLKSKLVSDFRKDFQFYKVREINNYHHAHDAYLNAVVGTALIKKYPKLESEFVYGDYKVYDVRKMIAKSEQEIGKATAKYFFYSNIMNFFKTEITLANGEIRKRPLIETNGETGEIVWDKGRDFATVRKVLSMPQVNIVKKTEVQTGGFSKESILPKRNSDKLIARKKDWDPKKYGGFDSPTVAYSVLVVAKVEKGKSKKLKSVKELLGITIMERSSFEKNPIDFLEAKGYKEVKKDLIIKLPKYSLFELENGRKRMLASAGELQKGNELALPSKYVNFLYLASHYEKLKGSPEDNEQKQLFVEQHKHYLDEIIEQISEFSKRVILADANLDKVLSAYNKHRDKPIREQAENIIHLFTLTNLGAPAAFKYFDTTIDRKRYTSTKEVLDATLIHQSITGLYETRIDLSQLGGDPKKKRKVEDPKKKRKVGGGGGMDAKSLTAWSRTLVTFKDVFVDFTREEWKLLDTAQQIVYRNVMLENYKNLVSLGYQLTKPDVILRLEKGEEP

SEQ ID NO: 81 - protein, 1367 aa, synthetic construct
DKKYSIGLAIGTNSVGWAVITDEYKVPSKKFKVLGNTDRHSIKKNLIGALLFDSGETAEATRLKRTARRRYTRRKNRICYLQEIFSNEMAKVDDSFFHRLEESFLVEEDKKHERHPIFGNIVDEVAYHEKYPTIYHLRKKLVDSTDKADLRLIYLALAHMIKFRGHFLIEGDLNPDNSDVDKLFIQLVQTYNQLFEENPINASGVDAKAILSARLSKSRRLENLIAQLPGEKKNGLFGNLIALSLGLTPNFKSNFDLAEDAKLQLSKDTYDDDLDNLLAQIGDQYADLFLAAKNLSDAILLSDILRVNTEITKAPLSASMIKRYDEHHQDLTLLKALVRQQLPEKYKEIFFDQSKNGYAGYIDGGASQEEFYKFIKPILEKMDGTEELLVKLNREDLLRKQRTFDNGSIPHQIHLGELHAILRRQEDFYPFLKDNREKIEKILTFRIPYYVGPLARGNSRFAWMTRKSEETITPWNFEEVVDKGASAQSFIERMTNFDKNLPNEKVLPKHSLLYEYFTVYNELTAVKYVTEGMRKPAFLSGEQKKAIVDLLFKTNRKVTVKQLKEDYFKKIECFDSVEISGVEDRFNASLGTYHDLLKIIKDKDFLDNEENEDILEDIVLTLTLFEDREMIEERLKTYAHLFDDKVMKQLKRRRYTGWGRLSRKLINGIRDKQSGKTILDFLKSDGFANANFMALIADDSLTFKEDIQKAQVSGQGDSLHEHIANLAGSPAIKKGILQTVKVVDELVKVMGRHKPENIVIEMARENQTTQKGQKNSRERMKRIEEGIKELGSQILKEHPVENTQLQNEKLYLYYLQNGRDMYVDQELDINRLSDYDVDAIVPQSFLKDDSIDNKVLTRSDKNRGKSDNVPSEEVVKKMKNYWRQLLNAKLITQRKFDNLTKAERGGLSELDKAGFIKRQLVETRQITKHVAQILDSRMNTKYDENDKLIREVKVITLKSKLVSDFRKDFQFYKVREINNYHHAHDAYLNAVVGTALIKKYPKLESEFVYGDYKVYDVRKMIAKSEQEIGKATAKYFFYSNIMNFFKTEITLANGEIRKRPLIETNGETGEIVWDKGRDFATVRKVLSMPQVNIVKKTEVQTGGFSKESILPKRNSDKLIARKKDWDPKKYGGFDSPTVAYSVLVVAKVEKGKSKKLKSVKELLGITIMERSSFEKNPIDFLEAKGYKEVKKDLIIKLPKYSLFELENGRKRMLASAGELQKGNELALPSKYVNFLYLASHYEKLKGSPEDNEQKQLFVEQHKHYLDEIIEQISEFSKRVILADANLDKVLSAYNKHRDKPIREQAENIIHLFTLTNLGAPAAFKYFDTTIDRKRYTSTKEVLDATLIHQSITGLYETRIDLSQLGGD

SEQ ID NO: 82 - protein, 544 aa, synthetic construct
MNHDQEFDPPKVYPPVPAEKRKPIRVLSLFDGIATGLLVLKDLGIQVDRYIASEVCEDSITVGMVRHQGKIMYVGDVRSVTQKHIQEWGPFDLVIGGSPCNDLSIVNPARKGLYEGTGRLFFEFYRLLHDARPKEGDDRPFFWLFENVVAMGVSDKRDISRFLESNPVMIDAKEVSAAHRARYFWGNLPGMNRPLASTVNDKLELQECLEHGRIAKFSKVRTITTRSNSIKQGKDQHFPVFMNEKEDILWCTEMERVFGFPVHYTDVSNMSRLARQRLLGRSWSVPVIRHLFAPLKEYFACVSSGNSNANSRGPSFSSGLVPLSLRGSHMGPMEIYKTVSAWKRQPVRVLSLFRNIDKVLKSLGFLESGSGSGGGTLKYVEDVTNVVRRDVEKWGPFDLVYGSTQPLGSSCDRCPGWYMFQFHRILQYALPRQESQRPFFWIFMDNLLLTEDDQETTTRFLQTEAVTLQDVRGRDYQNAMRVWSNIPGLKSKHAPLTPKEEEYLQAQVRSRSKLDAPKVDLLVKNCLLPLREYFKYFSQNSLPL

SEQ ID NO: 83 - protein, 302 aa, synthetic construct
MNHDQEFDPPKVYPPVPAEKRKPIRVLSLFDGIATGLLVLKDLGIQVDRYIASEVCEDSITVGMVRHQGKIMYVGDVRSVTQKHIQEWGPFDLVIGGSPCNDLSIVNPARKGLYEGTGRLFFEFYRLLHDARPKEGDDRPFFWLFENVVAMGVSDKRDISRFLESNPVMIDAKEVSAAHRARYFWGNLPGMNRPLASTVNDKLELQECLEHGRIAKFSKVRTITTRSNSIKQGKDQHFPVFMNEKEDILWCTEMERVFGFPVHYTDVSNMSRLARQRLLGRSWSVPVIRHLFAPLKEYFACV

SEQ ID NO: 84 - protein, 242 aa, synthetic construct
SSGNSNANSRGPSFSSGLVPLSLRGSHMGPMEIYKTVSAWKRQPVRVLSLFRNIDKVLKSLGFLESGSGSGGGTLKYVEDVTNVVRRDVEKWGPFDLVYGSTQPLGSSCDRCPGWYMFQFHRILQYALPRQESQRPFFWIFMDNLLLTEDDQETTTRFLQTEAVTLQDVRGRDYQNAMRVWSNIPGLKSKHAPLTPKEEEYLQAQVRSRSKLDAPKVDLLVKNCLLPLREYFKYFSQNSLPL

SEQ ID NO: 85 - protein, 80 aa, synthetic construct
GGPSSGAPPPSGGSPAGSPTSTEEGTSESATPESGPGTSTEPSEGSAPGSPAGSPTSTEEGTSTEPSEGSAPGTSTEPSE

SEQ ID NO: 86 - protein, 31 aa, synthetic construct
PKKKRKVEDPKKKRKVGGGGGMDAKSLTAWS

SEQ ID NO: 87 - protein, 62 aa, synthetic construct
RTLVTFKDVFVDFTREEWKLLDTAQQIVYRNVMLENYKNLVSLGYQLTKPDVILRLEKGEEP

SEQ ID NO: 88 - protein, 7 aa, synthetic construct
GGGSGGS

SEQ ID NO: 89 - protein, 5 aa, synthetic construct
SGGGS

SEQ ID NO: 90 - protein, 16 aa, synthetic construct
SGSETPGTSESATPES

SEQ ID NO: 91 - protein, 4 aa, synthetic construct
GGGS